European Patent Application EP 4 276 058 A1, published November 15, 2023. Title: AC-field driven macromolecular rotary motor. Applicant: Technische Universitaet Muenchen. The sequence listing filed with the application follows.

SEQUENCE LISTING (1125 sequences)

SEQ ID NO: 1 - DNA, 7585 bp, Artificial Sequence
  artificial sequence
agcttatatcctatggaatgagattgtaggactcaaaagttgaaagggagaggttaacaaggaggggtccctaggtcacactagggtataatgtgctagtggaccaagtcccatcatagtggagtatgtaggggatgatcccactgagtttgtgtgtcttctcctgaatacaacataccaggggacacttgcagggattgagacttagtgtctgtactggttcaccttcttcaactctcagacatttaccctggtgaccaattccctagagatagactgttaaatgatgaatcagtctatgataagaccttcccaagagaaggttgatagtcttaggtatccctagtcacttgtggatggttgcttgggttccacatccctcaaaatggggtagtcacaagagggttactcttgtctaaaccccactcaaaccttaaaggaagatttcctagactaccagatattacgtattttctgagttcttacccttaccagtcccaaaccctcaatgatatgtgagttgtcttgtacttggtcaggaccgactcctatatagggatctacaatgccctagaaggataagtctctggtactcacctagaaactaattctgaactcaactcccgttctttggtttgtggggttcattagtttggtcgtctatcacttgagaagacaagagttataaacttaaccacccagcaggatctgttcaaatcactaggctaaattccccacctaaggcaggaatccttgacagaactgaactggtttgagaattgcattgggaaaagaattttaacctaatgacgtgtggaaaactacaaatcataacatactggacactgtagtattactcacaggttcctgattctctcatctacccatccttttcaccggattgggtgcctggtcaaggggatcatcccatgggatggtgagggatgcttctttcaggggtaatgttagaaatgtacacatacctatagaatgagtctgaaattcagaaggaagttatcagttaaaacccctgatatttagttatgaggatgagttggttaatatactacatcaagtgtcacctctgactgtgtctgaacaggagtatcctaagatggtattaaacttgcatggaaataagtgaaatcaacatcaggtagtagtgaactaaaccagacttcatcaattatcaatactcgtacagggacaacttcccaggacatgtgtttactccccaaaagggtaaccgttggaccttctggacaggttatttcacctccttcttggagtcatctgactcagtgcagatgtaggtaggaacaatgaccacgtccgaaaggagtgttcactggattgtacaatcacaccgttctgatacagagtctaatacctagttggaggacattcatgtatcttttactagttttccttcaaacaatgggattaagtgacagtgtaacttccatttctgattggataactgtgttttgtgtatgggaaacacagaagatctaaaccggtttgttacccctgtaccacacttcatgatggtttggggagagtttactaaccagtctggagagtagaattaacactgtgagcgagggccctgtagttaggtttctcctagatctcctactggtggtggggtggaacaaattttactctcacttagtaaggtggacatcgaaaccactggcagtctaagccccacgtctgtttgactgtctggggaacaacactggttagacttatggtctggtggatagtagaactaatctcctgggtaccagtattggtccagtgtcctctgttaggagtaagctactcccaaagagtgagagtgtcagtctgtctgttgtcccttttgataaaagtataactttaccccaacaaagttggtcctgtgggcagtccatgaaaggtttattttgttccctgatcctcatgttttattgaggggttcttcataaggtattgacttggcaaatggagggtggtgatactagtgaaaccgatctgtaaggacctgtggaactcacactccataagtcaaccagaacttgaaagttagaggtctgggacgagtggggacagggcacaccggttttcagtgtgtagggagtaaactgtttggatttatcctctattttatccacagtgtgactgtatatggggtttccacaaagtcagtaggaatgatgggagaccaaggtcttctgtcactttataggtcctttgttcaccgattacaggaatgtaccaaggggtacatctactaggtcccctatagtattcccagattagaaaacacatggctctggactttatgcagacactcagggcctggtgtagtcagtgatgtcaactcaggcccttgtacactgttgatcaggaacctccatgttctgaggttctcttgcaccagggtttaagggagtttaagaatgaactcctgacttcctatctacacttatttacttcacttaaaacacccctcatctgttggggaaagaaggtgtattttgaggccttctccaaagaaatctaagaaaataggatgcccagtgaagtgtgaggtctcagatacccaggcccaatcttctcaagacatcaccattggtaagtgtggggattcattacctaggttctacaaacctagattctatgaaagtcattccaccccacccatgatcagataattgatagaatctgaaaggatagataccattacatggtactaagttggcaataccaataagtaggacacctttatgattataactggtccaagtggtccgggaattatctcttcttgtccccttcaggagagtgaaagtggtgttctgtcttggggtactggggttatggaggtatgactcaatcagatttcacatccatattgtgatatgggagcctagacaattaccctacaccagaggagatcatgacaactagaccaatatcatgaatcccacaagcatggtcaaatatgatgacagtccctatactatcagatcccattgaaactagaattcaacagttacaggtgttatgactgcaggctatatcatctggtaggtggtgtacttctgtattgatgttggtagggtactctccatcagtgggtccttattactatgtattgggtctggaccctgaaatctgagagatcactgtaatgggaaggtccaatcatctattcccctaattcactatcctagtcgtcagaggaaatcagtgacactactgattcagcctgttcacggtcggtcagagtcgtctgagaacccacaactcacttggaaggatggtaggaggttcagtagtacattcactgtgtactccctacctgatttcattcctatgtacattagaccccatgagacaactggaggattgaaaagcagtggggtcatgatcttgttgggtccaactgggattctggtgtttagaccagaccatgtaggagtcaatacatcagtcagttactcctaccctccaagtcttggtgatggactgaataaggtgatttctagtgatctccatacagatgcgaggggaacctattaagagtaaatccatagacagtactccatctccgagggaacagggatccaacgacaaaggagacctgcaaagatacctcattctatcctcggttgtatcccctgtgaaaggcactatatccatcttggacagtcaggttttgtcactcagtttaggtcagttggggtgtctggatgatagatcatctctctcacacctgaagccctgaatggttaggactgtaacacctagtgaccacctctagggaattggttagtagtataggaccttaagttgtataccttactacaatacactctgagtatgcccacaatcccaggtctgaagagatggagtctagtggtcaccttggtacttcaggtaaggagatagggacattaatctgtggatataggagggtcagcctaggtaactagtaccctatctgtctccgtgtccctgaggtgtcaaaagctccaacttggggatcccaacataacccttaggggtctgagggtccacaatagacataattgtaaaattccaggactcccattacttctataacatgacctctcccaaccacaaaccatattaagtatgacacattgggttacacatgatccacaagtgagtcaagttcactaatttcaagagactcaagttgtcaggtatcagacacatcttagtctgacccttgtcaaaccacctggaacatattatattgatcatcacaactatagttcaatgggtaaagaacctggaggggacccttttctgtacccatgtggttacctactcttaagggtacaggtctagttccttggttttggaccccacaggtagatttagtcaaaactttcctgtaatcctacttgtaaatatatacagctccctggttaaggtaagtctggtatgatggaaaccaggtaaacccaaaggactctttgatcacatcagaaccttttacctcacaatcttgataatataatacccctacttagggtctgtagtggataaagtgggtatcttacctttctcaatgttgaccagtaaggggtgagatagtttgattttcggattccctccccagatcaaacccatattctatagggtcaaccctttaaccggttgatgtcctaggacatatctcccatagaaaatccacacatagttctgaaggttaagtacttaacataggttccctctaagggttcaggcatataggtgttggttctgtggtcagaatcactccaagaaatggatctaaagtgatcgaaagggttaatctcacaacaccacccctggtccctgtgtcatgaaacactgaaccccaatgttacatcatgtcagtgtctacccttgctttaagtgttggaaacaagtccagtcacataatgtactcggaagtccaaagtgaggaaactttagaaagtttctcttcaatttaacaatgtcaccaagaactacttggacttgagtaacttatgccttgagtcttaatgtaggcatgagtcgttaccttggaaatgggaggtcattgtgtttcatatgacccaggtatggccggtgcagtccccgaaaaggtcatccggtctcaagtggggccatgacttagagtaagagtcctggtgggattggaacccagactgatatatgagagttgtgaaacaggaactggatccaccagtcgacctaagagatttaccttctacagacacccacatcaaaacagtacagaacatgctctaggacttagggcagtgtatccaccctcgtccccacacaaagggataacagacaatctccaccttccacttatctgtaggatcagagattggtcatggatccgggacccacaccaatcaactgttaccgaagtctatagatcctctctgtcatagtcccctcttgtgtgagagaaattcctcatcccttgttccattggggtctatatgttcatattactgactcctcagttgttgcatgtttgggatgttcttgaaataaatgactctcaagggacctgccttaggttggggctgaggtaggtaatgatctcatatcttgtcagttcatctaattgtgtctcaaccatgaatatgtgttccgtgactaaggggaaactgcctacctacagataaggggctccctctgatcaatatatcacctaaatgccacttttgttggactctctaacatggtccttgatgggtgggaactgtgaccatagtgttaaggaaccaaaagtaccatatggtgattcctttgatggattggtgtcgtcttcttcccgtccatccactagtgtaataatagaacccctaccaccaaatgggttgttttcttcaggcctctatcccacccttgatccccataattttagaggacaaactctggctcatgtgaagataggttttctgggtctttcccatataagacttcgttccttcctaaagaaaactgtactcaaataatccaccgacaggaaattgggtacaaggaaatactctgtcggatatcaatgagtacataaatacctcttagagggaatcaattcttaagatagatgtctacggtccagactcgacatgatgtcttgactgagtgtgaatagaatacacgtaacaggggtcaattagagttcaccccagagttgggttgactggatgtggaatgggtgtcagagacttctctctggatttgttctagacagaggtcggtggtttatgtccctcagatctactttggtcacgtagatacttgggaatcgaggtagacaggggatatggttacataggaagtgacctcaacctcttggttccatggggaattcccatctacatctgggaggagaagattgtgtagttctacttccaaaacgcaatctacagtgttttagcctttagtttacccaaactcccctgaccaggttcttataacactcatatgtaagggaatatcactcactccgagaagagaaaagactccttggggccctttattcagagagaggactcgatcatgttatctggggtcctattgacagggtggggaaggaacattctactgtatcctgggagtcaggaattcatactttaaggtccggtgggacagctggttcccaccattctctacatagtgaagaggattatctttcttccagacctcatcacttataggggaatccacggtgtccttagttttagacatccttctgtgaatgtctggttgtgagaatctcagttccccatccaaataccacatctcatcaactattcagtaagttagttcatagggtaagaacttaatatggtcacagggaatggtccactctctcttttcatgtgtacggacttgggcatgtacagtgagttccctatgttctcaggggaagtggattgatataagtgtaaacttcctggttggacattttcttgtgagtgatcaatgtatatccccaagatacaatggaagataagatatttcctggaatcatagaccacatgtgggtaagggtcccattctggatctcgatcctccattaccatgtcacaataatctcttgatcaaatacaagatgggttaaagaatcccctttacctgtgtggtgtggttcatccaatctctagatgaacatacagggtacccctcccttaagaaaggaactctacttgaagttgttccttacttaggtgggagttgtttgatatgacaagaaagtaaacagtgtcaatggtatccgtaaggcatcagtagagggtgagtaatgaaagaaacaaatggttcctaagttcctacaaccagtgagcagaaggtactgacatgtccagaggtgggtagagagtaccaaatcctcagacccctgcacctggtctaaatttcctccccttggtcttagtaggagagactactccttatgcaacctaggggtgggtgtggattctagttgtggaagttctaaccctcccaagtgaagggttggatagagtggaggagtccactgaaatggtaactgatgtggggcacacgttga

SEQ ID NO: 2 - DNA, 42 bp, Artificial Sequence
  artificial sequence
ggcattccacatccgtaggatccttcccgactcccccctaag

SEQ ID NO: 3 - DNA, 35 bp, Artificial Sequence
  artificial sequence
gtggatcgtgaattattagttggttaagtttataa

SEQ ID NO: 4 - DNA, 42 bp, Artificial Sequence
  artificial sequence
agaaccttaaagggccccaagtcttcacatagggtcagatta

SEQ ID NO: 5 - DNA, 41 bp, Artificial Sequence
  artificial sequence
tttacccattgaatcacttcgtagaacctcacttaatatgg

SEQ ID NO: 6 - DNA, 35 bp, Artificial Sequence
  artificial sequence
agacccctgagagtacaattaagggagcctcactt

SEQ ID NO: 7 - DNA, 35 bp, Artificial Sequence
  artificial sequence
ggagtccggaaatcgactaggggtcttactatcca

SEQ ID NO: 8 - DNA, 42 bp, Artificial Sequence
  artificial sequence
gaccccagaccttaccccaagccactagtactgaatacacat

SEQ ID NO: 9 - DNA, 42 bp, Artificial Sequence
  artificial sequence
acctcagttacctgtggtattcactgtagttatcttccattg

SEQ ID NO: 10 - DNA, 42 bp, Artificial Sequence
  artificial sequence
gacagagaggatctcctttgtacatctaatcataccagacca

SEQ ID NO: 11 - DNA, 35 bp, Artificial Sequence
  artificial sequence
tatctccggacacgcacaagtttcctttaaggttt

SEQ ID NO: 12 - DNA, 35 bp, Artificial Sequence
  artificial sequence
ataatccgagtcttatatgagtgttatagagtggg

SEQ ID NO: 13 - DNA, 42 bp, Artificial Sequence
  artificial sequence
agattctcccctgagggatatacattgatctgctctgaggat

SEQ ID NO: 14 - DNA, 35 bp, Artificial Sequence
  artificial sequence
tagttgaacttgggccttctctaattccgctccca

SEQ ID NO: 15 - DNA, 42 bp, Artificial Sequence
  artificial sequence
actagtttgtggaagtttagacaagagtcccttacttctctt

SEQ ID NO: 16 - DNA, 35 bp, Artificial Sequence
  artificial sequence
gagacagtatgtagagaatggctctgaaggtcagg

SEQ ID NO: 17 - DNA, 35 bp, Artificial Sequence
  artificial sequence
ttccctattcagggtccagaaggggattaaccgag

SEQ ID NO: 18 - DNA, 36 bp, Artificial Sequence
  artificial sequence
aactctatttggaactatgtaaccatattgaggttc

SEQ ID NO: 19 - DNA, 35 bp, Artificial Sequence
  artificial sequence
tgtgagaatactactggtctagcataaggtatatt

SEQ ID NO: 20 - DNA, 42 bp, Artificial Sequence
  artificial sequence
catggtagtatttgagtgcctttcacagggatcccaacaact

SEQ ID NO: 21 - DNA, 35 bp, Artificial Sequence
  artificial sequence
gtgatcattcacaacaggactcttactccaatgac

SEQ ID NO: 22 - DNA, 35 bp, Artificial Sequence
  artificial sequence
ctttaacccatcttatggaggcattgactcacctt

SEQ ID NO: 23 - DNA, 49 bp, Artificial Sequence
  artificial sequence
gatagaatgaggccaccacacaggtaaatgggaccctactgacaagact

SEQ ID NO: 24 - DNA, 42 bp, Artificial Sequence
  artificial sequence
ctttgggtttacaaagtcaactcttctcccaagaggttgagg

SEQ ID NO: 25 - DNA, 35 bp, Artificial Sequence
  artificial sequence
gacctggttcttacgaccattaggtcctgagatga

SEQ ID NO: 26 - DNA, 42 bp, Artificial Sequence
  artificial sequence
aacacttaaagcaatggacttagagggaagggtggaagtccg

SEQ ID NO: 27 - DNA, 35 bp, Artificial Sequence
  artificial sequence
cccacctcggatacatcgagacttcagggagtgat

SEQ ID NO: 28 - DNA, 35 bp, Artificial Sequence
  artificial sequence
aagtggattggtgtgagtcagacatcccacacata

SEQ ID NO: 29 - DNA, 49 bp, Artificial Sequence
  artificial sequence
tttacctactggtgtggccccacttgagatacctgtgttatcatagact

SEQ ID NO: 30 - DNA, 42 bp, Artificial Sequence
  artificial sequence
ccatcactgccttaaagtaagtctcctttgtcgttgggatac

SEQ ID NO: 31 - DNA, 49 bp, Artificial Sequence
  artificial sequence
aattatggacccagttgagaccatttatttcaagataatatgtacccac

SEQ ID NO: 32 - DNA, 42 bp, Artificial Sequence
  artificial sequence
gaggtggtgtattgactaagatcagaggctgaattattagac

SEQ ID NO: 33 - DNA, 42 bp, Artificial Sequence
  artificial sequence
agtaccttcactcaatatcaatccacttcacaaccagttacc

SEQ ID NO: 34 - DNA, 35 bp, Artificial Sequence
  artificial sequence
gtaggaatatcttggaacatagggaacttggatgg

SEQ ID NO: 35 - DNA, 42 bp, Artificial Sequence
  artificial sequence
cttaggatttagaccaggtgctggactcggaactgatgtccc

SEQ ID NO: 36 - DNA, 35 bp, Artificial Sequence
  artificial sequence
ttggtacccacatcagacattccctcctatatcca

SEQ ID NO: 37 - DNA, 35 bp, Artificial Sequence
  artificial sequence
gaggaaaacgtaactgactgatcactagcatgccc

SEQ ID NO: 38 - DNA, 35 bp, Artificial Sequence
  artificial sequence
gagtagtgaacttcactaactactccattctgggg

SEQ ID NO: 39 - DNA, 49 bp, Artificial Sequence
  artificial sequence
taggcagagagaaaaacattgcttttggttccttaagacgactttcttg

SEQ ID NO: 40 - DNA, 42 bp, Artificial Sequence
  artificial sequence
aacagtcacagaacacctccagagagaatcaggaaagttatc

SEQ ID NO: 41 - DNA, 49 bp, Artificial Sequence
  artificial sequence
gtctaatagaatccacacccatattaaggattgtgccctataactacag

SEQ ID NO: 42 - DNA, 35 bp, Artificial Sequence
  artificial sequence
tctgtactcattgatttatccgaatatgatcttca

SEQ ID NO: 43 - DNA, 28 bp, Artificial Sequence
  artificial sequence
attgcgtattgaccccaccgacctctgt

SEQ ID NO: 44 - DNA, 35 bp, Artificial Sequence
  artificial sequence
tatccgaaattcctcaccctgttgggagattagtg

SEQ ID NO: 45 - DNA, 35 bp, Artificial Sequence
  artificial sequence
cccaagcatcatttatttcagaggggtcactggtt

SEQ ID NO: 46 - DNA, 49 bp, Artificial Sequence
  artificial sequence
gatacctttttgaccagctgtatttcctaccgtaggtggggaggactgc

SEQ ID NO: 47 - DNA, 49 bp, Artificial Sequence
  artificial sequence
aagactatatctggaggagtcgtgtcacgcagtcacaccacctaccaga

SEQ ID NO: 48 - DNA, 35 bp, Artificial Sequence
  artificial sequence
ggagtacttgggataagtatgcagagtaaattgat

SEQ ID NO: 49 - DNA, 35 bp, Artificial Sequence
  artificial sequence
tagtctaaatgtgttgatcgactttaccttaacca

SEQ ID NO: 50 - DNA, 42 bp, Artificial Sequence
  artificial sequence
tacgtaatcggtagaatcaaaagggttactctcctactccta

SEQ ID NO: 51 - DNA, 35 bp, Artificial Sequence
  artificial sequence
aagaactacaagaccgtgaacgttgaataccaaca

SEQ ID NO: 52 - DNA, 42 bp, Artificial Sequence
  artificial sequence
ggtaagaaacatattcggtaacagttgaaggtggatccctct

SEQ ID NO: 53 - DNA, 35 bp, Artificial Sequence
  artificial sequence
accaagtcagaaaatttgtggtcaataggtatata

SEQ ID NO: 54 - DNA, 42 bp, Artificial Sequence
  artificial sequence
atcagtaggtcctgtgtctagcggaccacttcctttgacact

SEQ ID NO: 55 - DNA, 49 bp, Artificial Sequence
  artificial sequence
tgagaaaagggaattgggaaagggatcaacctatgtctgaccgatggac

SEQ ID NO: 56 - DNA, 35 bp, Artificial Sequence
  artificial sequence
ttggaccagaacggcttctcaagtgatagtaccct

SEQ ID NO: 57 - DNA, 35 bp, Artificial Sequence
  artificial sequence
ttcccatgaccgacaactcactctcctcaatcata

SEQ ID NO: 58 - DNA, 35 bp, Artificial Sequence
  artificial sequence
tcaacatgtacccacccaccggataacacatactt

SEQ ID NO: 59 - DNA, 35 bp, Artificial Sequence
  artificial sequence
aaaacctggtttgactcttcaggttatgacagtga

SEQ ID NO: 60 - DNA, 42 bp, Artificial Sequence
  artificial sequence
agaagtataacacctgcaattatttgtaatcaacatctgtat

SEQ ID NO: 61 - DNA, 35 bp, Artificial Sequence
  artificial sequence
tcaatacctcttgtgagttgagttcagaaggggaa

SEQ ID NO: 62 - DNA, 49 bp, Artificial Sequence
  artificial sequence
gatatattgatcaggatgaactcttataccgaaaaaaggtgattggagc

SEQ ID NO: 63 - DNA, 35 bp, Artificial Sequence
  artificial sequence
tctagttcagttaaaattcttcagtgttcattcct

SEQ ID NO: 64 - DNA, 42 bp, Artificial Sequence
  artificial sequence
ctatagtcatgggtacagaaactagaactggggtggggagct

SEQ ID NO: 65 - DNA, 42 bp, Artificial Sequence
  artificial sequence
tacacaaccaactcaaatccagagagaagtaaccatgtgatg

SEQ ID NO: 66 - DNA, 35 bp, Artificial Sequence
  artificial sequence
ttcccaatgtaactaggctgatagatgaaacttga

SEQ ID NO: 67 - DNA, 42 bp, Artificial Sequence
  artificial sequence
ctgtcattcaatggcgactcttacagtgttgagtcatgtaga

SEQ ID NO: 68 - DNA, 35 bp, Artificial Sequence
  artificial sequence
ctgccagagtttgtttcagaaagatccaaccaatc

SEQ ID NO: 69 - DNA, 35 bp, Artificial Sequence
  artificial sequence
cctctaagagagtgcctatgacacaactgtacata

SEQ ID NO: 70 - DNA, 28 bp, Artificial Sequence
  artificial sequence
cgagggtggactattgaggaacccaacc

SEQ ID NO: 71 - DNA, 42 bp, Artificial Sequence
  artificial sequence
cagttattggtgtaacacgtcattagtactcagaatgtacaa

SEQ ID NO: 72 - DNA, 28 bp, Artificial Sequence
  artificial sequence
cattaccaggaaaacaatcagaaatgga

SEQ ID NO: 73 - DNA, 49 bp, Artificial Sequence
  artificial sequence
gttttaagtgtgatcatggagggccctgtaaactcgaccataacagacg

SEQ ID NO: 74 - DNA, 35 bp, Artificial Sequence
  artificial sequence
atcagggaaccaactatctattaggtaaagtattg

SEQ ID NO: 75 - DNA, 35 bp, Artificial Sequence
  artificial sequence
gtgtacaagggctgtccagtatatcacacctatat

SEQ ID NO: 76 - DNA, 35 bp, Artificial Sequence
  artificial sequence
tcatcctcccacccctaggttaacaccactagaaa

SEQ ID NO: 77 - DNA, 42 bp, Artificial Sequence
  artificial sequence
tcaattaagaatctctggtttagttcacggtccaattctttg

SEQ ID NO: 78 - DNA, 49 bp, Artificial Sequence
  artificial sequence
ctttcattctgatctttccccacctacaggaaaacatgaggactttcat

SEQ ID NO: 79 - DNA, 35 bp, Artificial Sequence
  artificial sequence
aggtttgattcagtcatggtctaaccaagaaaaga

SEQ ID NO: 80 - DNA, 28 bp, Artificial Sequence
  artificial sequence
tagaacccctttcagttttaatcggacg

SEQ ID NO: 81 - DNA, 42 bp, Artificial Sequence
  artificial sequence
gatagagaacgaagtgacaagtaaggcaggtccctaatggaa

SEQ ID NO: 82 - DNA, 49 bp, Artificial Sequence
  artificial sequence
ataattggggagtagggcatcctattttgaggggtgattctatgatgta

SEQ ID NO: 83 - DNA, 42 bp, Artificial Sequence
  artificial sequence
ctgtacgtgaatccgagatcagaatccccaacttaccctgtg

SEQ ID NO: 84 - DNA, 35 bp, Artificial Sequence
  artificial sequence
gagaaggcctcaaataacctgtccagaatactacc

SEQ ID NO: 85 - DNA, 35 bp, Artificial Sequence
  artificial sequence
ttaagtaaagtttccccttatctgtaggttcatgg

SEQ ID NO: 86 - DNA, 42 bp, Artificial Sequence
  artificial sequence
gggaagaacactatcactgacatgatgtctttctacttaacc

SEQ ID NO: 87 - DNA, 35 bp, Artificial Sequence
  artificial sequence
caccttcatgggtggacacagccaagggacccttc

SEQ ID NO: 88 - DNA, 42 bp, Artificial Sequence
  artificial sequence
gggtagaggtcacagttcccaactagtgacagaacctaacca

SEQ ID NO: 89 - DNA, 49 bp, Artificial Sequence
  artificial sequence
atcaatacatggaactcccagtcttgaaaggtcattaagggtatgtact

SEQ ID NO: 90 - DNA, 35 bp, Artificial Sequence
  artificial sequence
gaacaacttcaagttcaccctcttaccctacagtc

SEQ ID NO: 91 - DNA, 42 bp, Artificial Sequence
  artificial sequence
tgttcctaacagatcttagatcggttacccttttgatgaagt

SEQ ID NO: 92 - DNA, 35 bp, Artificial Sequence
  artificial sequence
tggtcatcagaacgctgataacttggacggaatga

SEQ ID NO: 93 - DNA, 49 bp, Artificial Sequence
  artificial sequence
accggccaccggataatctcttaggtcgggtttcctcttaagtttcctt

SEQ ID NO: 94 - DNA, 42 bp, Artificial Sequence
  artificial sequence
ctagtaaaagatacgtgtacatcactctctgattcaaccatc

SEQ ID NO: 95 - DNA, 49 bp, Artificial Sequence
  artificial sequence
tccagctactaaataaggtgttcatgggactgaacctcagacaggatac

SEQ ID NO: 96 - DNA, 42 bp, Artificial Sequence
  artificial sequence
aaaacaccctgtgatctgattgagtcataccactttttctaa

SEQ ID NO: 97 - DNA, 42 bp, Artificial Sequence
  artificial sequence
ggagtgtctgaaaaccggtgttccaccatccccaatcgctca

SEQ ID NO: 98 - DNA, 35 bp, Artificial Sequence
  artificial sequence
actgtttacttttaattgtgatctatcatcacttt

SEQ ID NO: 99 - DNA, 35 bp, Artificial Sequence
  artificial sequence
gattgtcggtcatatgaaacataagtcagatccag

SEQ ID NO: 100 - DNA, 35 bp, Artificial Sequence
  artificial sequence
tcctgagttgacattgaagtggattagtccagtgg

SEQ ID NO: 101 - DNA, 28 bp, Artificial Sequence
  artificial sequence
accatcacactgacgaacccctcaatac

SEQ ID NO: 102 - DNA, 28 bp, Artificial Sequence
  artificial sequence
tggttagagtgtctgccaagtcaatacc

SEQ ID NO: 103 - DNA, 35 bp, Artificial Sequence
  artificial sequence
tggggctctcccatgtaatcggtgaacaagggccc

SEQ ID NO: 104 - DNA, 42 bp, Artificial Sequence
  artificial sequence
ttcctgtaagagtcaagaggtatttaaatacagatctcccat

SEQ ID NO: 105 - DNA, 35 bp, Artificial Sequence
  artificial sequence
cattcctactgactcagtcaaagtctaactacaca

SEQ ID NO: 106 - DNA, 35 bp, Artificial Sequence
  artificial sequence
ttgtggatgtaccccttggtaaattctactctcgg

SEQ ID NO: 107 - DNA, 49 bp, Artificial Sequence
  artificial sequence
tttcgatccagtgacagaagaccttggttagactgtctactagccctgt

SEQ ID NO: 108 - DNA, 18 bp, Artificial Sequence
  artificial sequence
aaataaactcagggaaca

SEQ ID NO: 109 - DNA, 28 bp, Artificial Sequence
  artificial sequence
gagttccacaggtctccatttgcataaa

SEQ ID NO: 110 - DNA, 56 bp, Artificial Sequence
  artificial sequence
ggactgcccacaggtcaaaagtctgcacactaggttcagactgaagagattgggaa

SEQ ID NO: 111 - DNA, 35 bp, Artificial Sequence
  artificial sequence
ttcaagtccccactcgtcccacccaggatggtaca

SEQ ID NO: 112 - DNA, 49 bp, Artificial Sequence
  artificial sequence
tctggttgacttatttatgaatacaccagttcctggttttccgggtaat

SEQ ID NO: 113 - DNA, 29 bp, Artificial Sequence
  artificial sequence
ggaatgatggagggtaggacatttgtttt

SEQ ID NO: 114 - DNA, 29 bp, Artificial Sequence
  artificial sequence
tttcttatccacgactaggataatgtgta

SEQ ID NO: 115 - DNA, 43 bp, Artificial Sequence
  artificial sequence
tttcacaagaggggatacactttttttgccctaagtcctaggg

SEQ ID NO: 116 - DNA, 33 bp, Artificial Sequence
  artificial sequence
atatgagtttaggtcattatgtgactaacattt

SEQ ID NO: 117 - DNA, 48 bp, Artificial Sequence
  artificial sequence
tttaaagtggcaatcattacctttttttacctcagctttctctcattt

SEQ ID NO: 118 - DNA, 38 bp, Artificial Sequence
  artificial sequence
tttgtccggacttgtttccaggaccatgttagagattt

SEQ ID NO: 119 - DNA, 29 bp, Artificial Sequence
  artificial sequence
tttgtaggggttctattattaccccatca

SEQ ID NO: 120 - DNA, 47 bp, Artificial Sequence
  artificial sequence
ctccacttcatagacctgaagtgtgaaagtaataccaaggattcttt

SEQ ID NO: 121 - DNA, 29 bp, Artificial Sequence
  artificial sequence
tttcaacccagcctgaacccttccgagta

SEQ ID NO: 122 - DNA, 30 bp, Artificial Sequence
  artificial sequence
ttttctttaggaagggcctgaagaaaattt

SEQ ID NO: 123 - DNA, 38 bp, Artificial Sequence
  artificial sequence
tttgatttgaacagatccttggaatttagcctagtttt

SEQ ID NO: 124 - DNA, 30 bp, Artificial Sequence
  artificial sequence
ttttgtcgagtctgggtcggtggattattt

SEQ ID NO: 125 - DNA, 29 bp, Artificial Sequence
  artificial sequence
tttattctattcacagtcctcttgggaac

SEQ ID NO: 126 - DNA, 30 bp, Artificial Sequence
  artificial sequence
tttgagggacataaacctgttacgtgtttt

SEQ ID NO: 127 - DNA, 36 bp, Artificial Sequence
  artificial sequence
tttttgggagtagcttactccctctaactaacagac

SEQ ID NO: 128 - DNA, 29 bp, Artificial Sequence
  artificial sequence
tttgcattgtagatcatatggagggacaa

SEQ ID NO: 129 - DNA, 43 bp, Artificial Sequence
  artificial sequence
agaaacccagttcaatagccttgatttcctctgttctaggttt

SEQ ID NO: 130 - DNA, 40 bp, Artificial Sequence
  artificial sequence
tttttcccaagtatctacgcccctgtactgtagacttggg

SEQ ID NO: 131 - DNA, 36 bp, Artificial Sequence
  artificial sequence
taaactaaattttttggctaaaacctacctcgattt

SEQ ID NO: 132 - DNA, 45 bp, Artificial Sequence
  artificial sequence
ctcggagggtctggctgtggattcccctatttttttaagtgatga

SEQ ID NO: 133 - DNA, 52 bp, Artificial Sequence
  artificial sequence
tttaaactaaggacaccgacacagaatacacttcaagaaaatgtccaacttt

SEQ ID NO: 134 - DNA, 36 bp, Artificial Sequence
  artificial sequence
tgagatgaagtacctcaaactatctcacagtttttt

SEQ ID NO: 135 - DNA, 33 bp, Artificial Sequence
  artificial sequence
acatgtggaaccacctgtatgttcatctagttt

SEQ ID NO: 136 - DNA, 43 bp, Artificial Sequence
  artificial sequence
tttagattggatgtctatgattttttttccaggaaatatctgt

SEQ ID NO: 137 - DNA, 50 bp, Artificial Sequence
  artificial sequence
tgttatgctcaaactaactacaaggacctataaaccccaccaccagtttt

SEQ ID NO: 138 - DNA, 30 bp, Artificial Sequence
  artificial sequence
tttttctttcattacagagttcctttcttt

SEQ ID NO: 139 - DNA, 43 bp, Artificial Sequence
  artificial sequence
ttttggaccaatttactaagtttttttgagagtaaaatttgtt

SEQ ID NO: 140 - DNA, 30 bp, Artificial Sequence
  artificial sequence
tttaggagatctaggggggtaacaaacttt

SEQ ID NO: 141 - DNA, 29 bp, Artificial Sequence
  artificial sequence
tgtttcctcctccatgagtcagatgattt

SEQ ID NO: 142 - DNA, 31 bp, Artificial Sequence
  artificial sequence
ttttgaaaggaggttttttctccaagaaata

SEQ ID NO: 143 - DNA, 27 bp, Artificial Sequence
  artificial sequence
ttttaaagttatcactctcactctttt

SEQ ID NO: 144 - DNA, 37 bp, Artificial Sequence
  artificial sequence
aaggatgagttacactgtcttttttacttaatcccat

SEQ ID NO: 145 - DNA, 33 bp, Artificial Sequence
  artificial sequence
tttctgccttaggtgggatgttctgttacagtg

SEQ ID NO: 146 - DNA, 48 bp, Artificial Sequence
  artificial sequence
tttcggtttagatctagactgaacttttaaccaactttgttggggttt

SEQ ID NO: 147 - DNA, 38 bp, Artificial Sequence
  artificial sequence
ttttcccatgggatgattagaagcatccctcaccattt

SEQ ID NO: 148 - DNA, 36 bp, Artificial Sequence
  artificial sequence
ggtagattaaccccagccccttgaccaggcaccttt

SEQ ID NO: 149 - DNA, 30 bp, Artificial Sequence
  artificial sequence
ttttcaacgtgtgcctctctacccaccttt

SEQ ID NO: 150 - DNA, 37 bp, Artificial Sequence
  artificial sequence
ttttttgatgtgggtgtctgtagtcaagacatcattt

SEQ ID NO: 151 - DNA, 33 bp, Artificial Sequence
  artificial sequence
cattctactgttcaggtttaataccatcttttt

SEQ ID NO: 152 - DNA, 38 bp, Artificial Sequence
  artificial sequence
ttttatttccatgcaaggttgatgttgatttcactttt

SEQ ID NO: 153 - DNA, 33 bp, Artificial Sequence
  artificial sequence
tttaggatactctaggtatatgaatgcatacac

SEQ ID NO: 154 - DNA, 36 bp, Artificial Sequence
  artificial sequence
gaaggtagaccttttcagcatgttctgtactgtttt

SEQ ID NO: 155 - DNA, 37 bp, Artificial Sequence
  artificial sequence
tttactaccccatttagggaattggtcaccagggtaa

SEQ ID NO: 156 - DNA, 27 bp, Artificial Sequence
  artificial sequence
tttgtatagggagaatactataggttt

SEQ ID NO: 157 - DNA, 33 bp, Artificial Sequence
  artificial sequence
ttccaagatcccacctctcatatatcagtcttt

SEQ ID NO: 158 - DNA, 27 bp, Artificial Sequence
  artificial sequence
ttttgggttccagtaacgactcatttt

SEQ ID NO: 159 - DNA, 37 bp, Artificial Sequence
  artificial sequence
ttttcaaggcataagttactacaccctaagtaggttt

SEQ ID NO: 160 - DNA, 27 bp, Artificial Sequence
  artificial sequence
tttaagtagtaggacatcaaccggttt

SEQ ID NO: 161 - DNA, 36 bp, Artificial Sequence
  artificial sequence
aactgaggggtcccggatccatgaccttaagacttt

SEQ ID NO: 162 - DNA, 44 bp, Artificial Sequence
  artificial sequence
tttcgcatctgtatgccacactgtaccattgtagataggaattt

SEQ ID NO: 163 - DNA, 27 bp, Artificial Sequence
  artificial sequence
tttgacattgtttggattttctatttt

SEQ ID NO: 164 - DNA, 43 bp, Artificial Sequence
  artificial sequence
tcggagatggatatatcaagagagacctaaactgagtgacttt

SEQ ID NO: 165 - DNA, 30 bp, Artificial Sequence
  artificial sequence
tttaaccctggtgcagtccagagccatttt

SEQ ID NO: 166 - DNA, 37 bp, Artificial Sequence
  artificial sequence
tttccaggggtggtgttcaccaggaatgtgagatttt

SEQ ID NO: 167 - DNA, 36 bp, Artificial Sequence
  artificial sequence
tttgggtatctgagacctcacaaaataaggtaatgg

SEQ ID NO: 168 - DNA, 43 bp, Artificial Sequence
  artificial sequence
catcaaatatggtagggttcagtgtttcatgacacagggattt

SEQ ID NO: 169 - DNA, 27 bp, Artificial Sequence
  artificial sequence
ttttaaccctttcgatccagacacttt

SEQ ID NO: 170 - DNA, 36 bp, Artificial Sequence
  artificial sequence
cttcactaacacatgtcctgggaagttgggcctttt

SEQ ID NO: 171 - DNA, 33 bp, Artificial Sequence
  artificial sequence
ctatgtgaaattgatttcccctttcttggtttt

SEQ ID NO: 172 - DNA, 38 bp, Artificial Sequence
  artificial sequence
tttactagtatcaccaccccttacagatcggtttcttt

SEQ ID NO: 173 - DNA, 37 bp, Artificial Sequence
  artificial sequence
taccaatggtgatttttttgtcttgagaagattgtcc

SEQ ID NO: 174 - DNA, 27 bp, Artificial Sequence
  artificial sequence
ttttggtatttataaactcccttattt

SEQ ID NO: 175 - DNA, 27 bp, Artificial Sequence
  artificial sequence
tttgtgttttctaattggataaatttt

SEQ ID NO: 176 - DNA, 30 bp, Artificial Sequence
  artificial sequence
tttaaaggttctgataagttttgactattt

SEQ ID NO: 177 - DNA, 29 bp, Artificial Sequence
  artificial sequence
ttttagtaataaggacccactgatggaga

SEQ ID NO: 178 - DNA, 29 bp, Artificial Sequence
  artificial sequence
gacgaccaaactccagacccaatacattt

SEQ ID NO: 179 - DNA, 33 bp, Artificial Sequence
  artificial sequence
catgaagtcacggaaaacatgcacaagtccttt

SEQ ID NO: 180 - DNA, 27 bp, Artificial Sequence
  artificial sequence
tttttaaagggttgaggcatactcttt

SEQ ID NO: 181 - DNA, 43 bp, Artificial Sequence
  artificial sequence
tttggtcagactaagatgtgggaattccctaatatgaccctta

SEQ ID NO: 182 - DNA, 27 bp, Artificial Sequence
  artificial sequence
ttttgggttctcagagatctgatattt

SEQ ID NO: 183 - DNA, 43 bp, Artificial Sequence
  artificial sequence
tttttccaaggtttgggactgggttataggaatgtttacagga

SEQ ID NO: 184 - DNA, 29 bp, Artificial Sequence
  artificial sequence
tttctgtggataaaatagagttccccaga

SEQ ID NO: 185 - DNA, 27 bp, Artificial Sequence
  artificial sequence
tttcctccagttgtccctacttatttt

SEQ ID NO: 186 - DNA, 27 bp, Artificial Sequence
  artificial sequence
tttggtattatattaagatgtctattt

SEQ ID NO: 187 - DNA, 43 bp, Artificial Sequence
  artificial sequence
agagaactttgaccgtcatgaatatcattgaggtgagttgttt

SEQ ID NO: 188 - DNA, 37 bp, Artificial Sequence
  artificial sequence
tttaaaacctgactgtccaagatggagtactgtcttt

SEQ ID NO: 189 - DNA, 27 bp, Artificial Sequence
  artificial sequence
tttcccaactttataggttcccctttt

SEQ ID NO: 190 - DNA, 33 bp, Artificial Sequence
  artificial sequence
tttccaaacagtttactccccagtgtctcagac

SEQ ID NO: 191 - DNA, 27 bp, Artificial Sequence
  artificial sequence
ttttaaggtataagttggacccaattt

SEQ ID NO: 192 - DNA, 27 bp, Artificial Sequence
  artificial sequence
tttagagtgtcactgcttttcaatttt

SEQ ID NO: 193 - DNA, 27 bp, Artificial Sequence
  artificial sequence
tttaatctacctgtgtgtctgatattt

SEQ ID NO: 194 - DNA, 36 bp, Artificial Sequence
  artificial sequence
agagtaggtctctgacaccgtccaaaaccaaggttt

SEQ ID NO: 195 - DNA, 37 bp, Artificial Sequence
  artificial sequence
tttaactagacctgtttccaggtggtttgacaagttt

SEQ ID NO: 196 - DNA, 38 bp, Artificial Sequence
  artificial sequence
tttggaattttacaatttaaagtaatgggagtcctttt

SEQ ID NO: 197 - DNA, 29 bp, Artificial Sequence
  artificial sequence
ttttcagggtaatgaaccccacaaaccaa

SEQ ID NO: 198 - DNA, 54 bp, Artificial Sequence
  artificial sequence
agggtcccctccaccaaagtagatctttttgacgatccatcgcccagggcgctg

SEQ ID NO: 199 - DNA, 62 bp, Artificial Sequence
  artificial sequence
gctgggttctaggtgagtaccagagattttgatcggtccgcggtgcggggaacgccactggc

SEQ ID NO: 200 - DNA, 51 bp, Artificial Sequence
  artificial sequence
aagtttgagcccgcccactcgtgcaattttgatattaaccctcttgtgttt

SEQ ID NO: 201 - DNA, 40 bp, Artificial Sequence
  artificial sequence
tttcaatccggtgaattttcgtagacagcaccgcgtgcgt

SEQ ID NO: 202 - DNA, 64 bp, Artificial Sequence
  artificial sequence
gtccaccactggtagactaacagaggacactttctgagtcgctctctcgcaacagaggtacctc

SEQ ID NO: 203 - DNA, 54 bp, Artificial Sequence
  artificial sequence
gtgacgatagaggtcatcatatccttttttaagggaggggtatatctttgcagg

SEQ ID NO: 204 - DNA, 59 bp, Artificial Sequence
  artificial sequence
taacacgaaagcaccggttaagcaaaatttttgtttgacctgaaaccccaagtatctct

SEQ ID NO: 205 - DNA, 38 bp, Artificial Sequence
  artificial sequence
ttttctggacatgtcttttaacattagcactcacgacc

SEQ ID NO: 206 - DNA, 39 bp, Artificial Sequence
  artificial sequence
caacacctatattttggtgttttgtttacaagcggtggc

SEQ ID NO: 207 - DNA, 54 bp, Artificial Sequence
  artificial sequence
tcacccttagatacgtgcgaaaaatttttttgagtaccccttactggcaaggga

SEQ ID NO: 208 - DNA, 44 bp, Artificial Sequence
  artificial sequence
tatgcggcgattgagtcaggtttttggaagttggatgtctattt

SEQ ID NO: 209 - DNA, 44 bp, Artificial Sequence
  artificial sequence
tgagggaacctaggaagaaagttttttcaccgcgccacatagca

SEQ ID NO: 210 - DNA, 52 bp, Artificial Sequence
  artificial sequence
atgcggccttcgtcgtttgcctacaaatctctgatccgattgtgaggtattt

SEQ ID NO: 211 - DNA, 52 bp, Artificial Sequence
  artificial sequence
atgcggccttcgtcgtttggacctagtagaaaccccatatacagtcacattt

SEQ ID NO: 212 - DNA, 51 bp, Artificial Sequence
  artificial sequence
atgcggccttcgtcgttttatggatttactctcttgtcatatcatgttccc

SEQ ID NO: 213 - DNA, 51 bp, Artificial Sequence
  artificial sequence
atgcggccttcgtcgtttgtcaggagttcatttgaacactccttgtgaagt

SEQ ID NO: 214 - DNA, 42 bp, Artificial Sequence
  artificial sequence
atgcggccttcgtcgtttcctgacaacatctctcagattttt

SEQ ID NO: 215 - DNA, 53 bp, Artificial Sequence
  artificial sequence
atgcggccttcgtcgttttgatattggtctagttatgcttgtgggattcattt

SEQ ID NO: 216 - DNA, 42 bp, Artificial Sequence
  artificial sequence
atgcggccttcgtcgtttcaagatcatgaccagccaactttt

SEQ ID NO: 217 - DNA, 42 bp, Artificial Sequence
  artificial sequence
atgcggccttcgtcgtttgggagatatgtcacattgtagttt

SEQ ID NO: 218 - DNA, 42 bp, Artificial Sequence
  artificial sequence
atgcggccttcgtcgtttttgtggaccctcctaccatccttt

SEQ ID NO: 219 - DNA, 22 bp, Artificial Sequence
  artificial sequence
actccactatgcagtgggatca

SEQ ID NO: 220 - DNA, 35 bp, Artificial Sequence
  artificial sequence
atgggacttggtccagagttgaatccctgcctcat

SEQ ID NO: 221 - DNA, 38 bp, Artificial Sequence
  artificial sequence
tccatagtttataagcttctgactagcatagccctttc

SEQ ID NO: 222 - DNA, 32 bp, Artificial Sequence
  artificial sequence
gtgtcccctggtataagtctcaagaaggtgaa

SEQ ID NO: 223 - DNA, 32 bp, Artificial Sequence
  artificial sequence
cactgttgtatacacacaaactccttgttaac

SEQ ID NO: 224 - DNA, 33 bp, Artificial Sequence
  artificial sequence
tcctacaataactcttgtgacctagggacccct

SEQ ID NO: 225 - DNA, 38 bp, Artificial Sequence
  artificial sequence
atgttgaatactctgggtgagcaaaaacaggacccaac

SEQ ID NO: 226 - DNA, 31 bp, Artificial Sequence
  artificial sequence
tatcatttctccccaacaaagaagttagctg

SEQ ID NO: 227 - DNA, 39 bp, Artificial Sequence
  artificial sequence
cgcaataaacaggaatcggggaataagggcgacacggaa

SEQ ID NO: 228 - DNA, 32 bp, Artificial Sequence
  artificial sequence
cggagttgaacagtgtgcgcaagtaagagttt

SEQ ID NO: 229 - DNA, 32 bp, Artificial Sequence
  artificial sequence
ggcaaaatgccgcaaaaaaaagaacccggcat

SEQ ID NO: 230 - DNA, 32 bp, Artificial Sequence
  artificial sequence
aaaagaggcagagcgaccccgttctggtcatg

SEQ ID NO: 231 - DNA, 52 bp, Artificial Sequence
  artificial sequence
acaggtgattagacgtatattttggccaatagcacaaccacaaagcatcgat

SEQ ID NO: 232 - DNA, 41 bp, Artificial Sequence
  artificial sequence
tatttcgttggcacctatgtggggcgctgtgtgcacgaacc

SEQ ID NO: 233 - DNA, 40 bp, Artificial Sequence
  artificial sequence
tgtggattccttatccagcagccaattacgcgacaaacca

SEQ ID NO: 234 - DNA, 32 bp, Artificial Sequence
  artificial sequence
ctagaccgaagtattgtctcagcgagattatc

SEQ ID NO: 235 - DNA, 52 bp, Artificial Sequence
  artificial sequence
ctgtcttggcatatcacgaatgatgcgttgccttgaattagctacgattcac

SEQ ID NO: 236 - DNA, 36 bp, Artificial Sequence
  artificial sequence
tttccagactcgactaccatcttcaggcccgttgta

SEQ ID NO: 237 - DNA, 40 bp, Artificial Sequence
  artificial sequence
ccgctggtagcggtggaaaaagagaggattagcccttgat

SEQ ID NO: 238 - DNA, 40 bp, Artificial Sequence
  artificial sequence
tagttgtcgcaccattggcttgggggccacgcagccaaag

SEQ ID NO: 239 - DNA, 47 bp, Artificial Sequence
  artificial sequence
ccgatttaaaggagcacccggtaaactcacatcttgatccgggctta

SEQ ID NO: 240 - DNA, 48 bp, Artificial Sequence
  artificial sequence
tcctggcgccttacaacagaaaaaaaggatcttctgacgctcgtcttg

SEQ ID NO: 241 - DNA, 32 bp, Artificial Sequence
  artificial sequence
aaaaaggagaggattcggcggtgctctgctga

SEQ ID NO: 242 - DNA, 40 bp, Artificial Sequence
  artificial sequence
ccgcctttgtgaatataagagattaggtatagaggactcg

SEQ ID NO: 243 - DNA, 40 bp, Artificial Sequence
  artificial sequence
ggtatgtaaaccgtttacttattttgtttgcaagggattt

SEQ ID NO: 244 - DNA, 40 bp, Artificial Sequence
  artificial sequence
gatcatctgatgtttgatcagcacagtctcgatgtaccgt

SEQ ID NO: 245 - DNA, 36 bp, Artificial Sequence
  artificial sequence
gggggtgcaacacggctcccccaaggccaattatga

SEQ ID NO: 246 - DNA, 44 bp, Artificial Sequence
  artificial sequence
ccagtaagctgaaggggcctaccatgtcgcgccggttcggccct

SEQ ID NO: 247 - DNA, 32 bp, Artificial Sequence
  artificial sequence
cgtaggtaatcctttggcacacctaccccatc

SEQ ID NO: 248 - DNA, 29 bp, Artificial Sequence
  artificial sequence
ctaaacgcgatgttgccgtggagcttatc

SEQ ID NO: 249 - DNA, 45 bp, Artificial Sequence
  artificial sequence
tacagcggagccagatcctgagagctctccttaaggatcggacat

SEQ ID NO: 250 - DNA, 48 bp, Artificial Sequence
  artificial sequence
tgaagtgaccgggatttgaacgttactgctaggacagagaaactgtcc

SEQ ID NO: 251 - DNA, 47 bp, Artificial Sequence
  artificial sequence
gtcgctgtgcatttattaactagtgcaggcttagggcccaatctgtc

SEQ ID NO: 252 - DNA, 45 bp, Artificial Sequence
  artificial sequence
aaattccctgaccggatacgatcaatcctgtgcgcgccatggatc

SEQ ID NO: 253 - DNA, 40 bp, Artificial Sequence
  artificial sequence
tcctaggtaaaagacttcgttgttgacccaccctacgccc

SEQ ID NO: 254 - DNA, 40 bp, Artificial Sequence
  artificial sequence
agacggaatgtagagcagttcaaaggaagggataacccaa

SEQ ID NO: 255 - DNA, 32 bp, Artificial Sequence
  artificial sequence
agccagttaccttcggtttgtacacactttac

SEQ ID NO: 256 - DNA, 48 bp, Artificial Sequence
  artificial sequence
acgaaaactcacgttaagcagcagctggtaacttggtagctagctgtg

SEQ ID NO: 257 - DNA, 32 bp, Artificial Sequence
  artificial sequence
aactataacaacccagcgtcagcttgaagcaa

SEQ ID NO: 258 - DNA, 48 bp, Artificial Sequence
  artificial sequence
gacttacaacttatcgctatatcagtcttatggcgagaaacgaggttc

SEQ ID NO: 259 - DNA, 40 bp, Artificial Sequence
  artificial sequence
cgctgctttactgttggagatacccatcgaatgtcggcta

SEQ ID NO: 260 - DNA, 40 bp, Artificial Sequence
  artificial sequence
tggagactccgggcatcctagtatgtataatcatcttttc

SEQ ID NO: 261 - DNA, 48 bp, Artificial Sequence
  artificial sequence
ccgcatccacctattttgaggcctattcggatgatgctcgtgtccgta

SEQ ID NO: 262 - DNA, 40 bp, Artificial Sequence
  artificial sequence
agtccaactttgtgtctacacagtacggggaaagccggcg

SEQ ID NO: 263 - DNA, 48 bp, Artificial Sequence
  artificial sequence
tcggcgtatactctcgtcagacgatagtggcatctatagcagtgtaca

SEQ ID NO: 264 - DNA, 37 bp, Artificial Sequence
  artificial sequence
tacggggcaagaagagacacgggatgtaagctaataa

SEQ ID NO: 265 - DNA, 54 bp, Artificial Sequence
  artificial sequence
ttaattctccgggcgcgctgcgtgtgtttggatccagtgggcgctaccgtctca

SEQ ID NO: 266 - DNA, 55 bp, Artificial Sequence
  artificial sequence
ttcggatacatatttgggagccctgatcttcccgctgttgagatccagttcgatg

SEQ ID NO: 267 - DNA, 36 bp, Artificial Sequence
  artificial sequence
tttgagattctgggtaagttagaaataccataagtt

SEQ ID NO: 268 - DNA, 35 bp, Artificial Sequence
  artificial sequence
ttcttcctttttcaatattttctgtgacatacttt

SEQ ID NO: 269 - DNA, 30 bp, Artificial Sequence
  artificial sequence
tggcggccgtgaattgccggccgaaacatt

SEQ ID NO: 270 - DNA, 37 bp, Artificial Sequence
  artificial sequence
agcccgacagtattacagggttattgtctcatgagtt

SEQ ID NO: 271 - DNA, 40 bp, Artificial Sequence
  artificial sequence
cccacgaaagttctgacgactgaccgtgtctgctcgtgca

SEQ ID NO: 272 - DNA, 47 bp, Artificial Sequence
  artificial sequence
aaacaagtgttcttattgacgtagcagccccgctgtaacgcgattgg

SEQ ID NO: 273 - DNA, 40 bp, Artificial Sequence
  artificial sequence
caacggtcttccacattgaggtattactaaaactgcgact

SEQ ID NO: 274 - DNA, 32 bp, Artificial Sequence
  artificial sequence
aagatgcctccgcactatattctcatatagac

SEQ ID NO: 275 - DNA, 29 bp, Artificial Sequence
  artificial sequence
tctgggactgctaaggtcgtggtatcaat

SEQ ID NO: 276 - DNA, 53 bp, Artificial Sequence
  artificial sequence
gtccttagggggcacgtgaaaactgtaccggtcaagacgcaacccgcgcgaga

SEQ ID NO: 277 - DNA, 48 bp, Artificial Sequence
  artificial sequence
tagaggtgtaaggttatcacaagttcatcgacagttcacaccagtgcc

SEQ ID NO: 278 - DNA, 40 bp, Artificial Sequence
  artificial sequence
aagtgccctcccaacggccgggagactcgaacatgcatca

SEQ ID NO: 279 - DNA, 47 bp, Artificial Sequence
  artificial sequence
gtttctcatagctatctaactattgcacacgggggttcattacagct

SEQ ID NO: 280 - DNA, 40 bp, Artificial Sequence
  artificial sequence
gccgttccctaaattcgaaattgggtcggcatgtgcgcct

SEQ ID NO: 281 - DNA, 31 bp, Artificial Sequence
  artificial sequence
gcgggcagtcaccccgtttcctctaaccgtg

SEQ ID NO: 282 - DNA, 48 bp, Artificial Sequence
  artificial sequence
gcctgtggcagtacgaatgacatacagttacccttacggtgatcagag

SEQ ID NO: 283 - DNA, 48 bp, Artificial Sequence
  artificial sequence
ctaacgactatgcttgaagtgtcatccatggtgggcttaccgtcccag

SEQ ID NO: 284 - DNA, 48 bp, Artificial Sequence
  artificial sequence
catttcgcgggccagaataaaaccatgcggcgttaactgatggagcga

SEQ ID NO: 285 - DNA, 40 bp, Artificial Sequence
  artificial sequence
gcaacgaaacttgacagacctcggagtgagtggggtgcag

SEQ ID NO: 286 - DNA, 40 bp, Artificial Sequence
  artificial sequence
tccgagttgttattaccacgataagagtctagccattagg

SEQ ID NO: 287 - DNA, 47 bp, Artificial Sequence
  artificial sequence
cgtatggttccaatgcggcagtcgcctgagtgtacgatcgctcgccg

SEQ ID NO: 288 - DNA, 56 bp, Artificial Sequence
  artificial sequence
gatagtgactcgatatgcatatgtcgatcattccttattgcgtacttttatcctgc

SEQ ID NO: 289 - DNA, 48 bp, Artificial Sequence
  artificial sequence
cgttaccggaggaggggatgcgaccatccattcacaacttaggtttgg

SEQ ID NO: 290 - DNA, 40 bp, Artificial Sequence
  artificial sequence
aagtcagaaaccgagcggatggagtgttatttgtcgccga

SEQ ID NO: 291 - DNA, 37 bp, Artificial Sequence
  artificial sequence
ggcctggacaactggccgagggctgtgtccaggtgct

SEQ ID NO: 292 - DNA, 56 bp, Artificial Sequence
  artificial sequence
agaaggcgacgggttaatacatgtgttatgcctgctcaccatgggctgatgtacaa

SEQ ID NO: 293 - DNA, 45 bp, Artificial Sequence
  artificial sequence
ttagttaggacctccttatcgacatccgggaggggttacgcctcc

SEQ ID NO: 294 - DNA, 40 bp, Artificial Sequence
  artificial sequence
aaacactaaaagttcgcacagcctgtggcctaaatagaag

SEQ ID NO: 295 - DNA, 38 bp, Artificial Sequence
  artificial sequence
actgacgttacggagtttgacactcttgatccctcaga

SEQ ID NO: 296 - DNA, 36 bp, Artificial Sequence
  artificial sequence
tataaggtgaagaccctcatgacgataggcactagc

SEQ ID NO: 297 - DNA, 32 bp, Artificial Sequence
  artificial sequence
aggctggctgacaccttatgctcaccataaca

SEQ ID NO: 298 - DNA, 37 bp, Artificial Sequence
  artificial sequence
ggaaagttagatcggcctgtcacgtttttggcggaat

SEQ ID NO: 299 - DNA, 32 bp, Artificial Sequence
  artificial sequence
taaggggtcctcaccgtcacgtgctgattcta

SEQ ID NO: 300 - DNA, 32 bp, Artificial Sequence
  artificial sequence
gagtggagcggaatctggtagctgctgcccaa

SEQ ID NO: 301 - DNA, 48 bp, Artificial Sequence
  artificial sequence
gagagcgcgttggttgttaggcctgaaaccgccgcgctgaaatgtttc

SEQ ID NO: 302 - DNA, 40 bp, Artificial Sequence
  artificial sequence
acgagtcagcacagtaagtccgaccggaaggtacccctag

SEQ ID NO: 303 - DNA, 40 bp, Artificial Sequence
  artificial sequence
ctccgcgagttttctccctaactctggataacggaaaaca

SEQ ID NO: 304 - DNA, 40 bp, Artificial Sequence
  artificial sequence
aatagcttataaatgttacctgttaacaccgcgcaaaggt

SEQ ID NO: 305 - DNA, 40 bp, Artificial Sequence
  artificial sequence
ggacgtaccctgccaggttaggctaagttcagacacggct

SEQ ID NO: 306 - DNA, 55 bp, Artificial Sequence
  artificial sequence
tgaacggatcggataaacgctcgatcctctaggctgtttattacgtgctgacgat

SEQ ID NO: 307 - DNA, 24 bp, Artificial Sequence
  artificial sequence
tcgcgacgtgtatacgtactcatc

SEQ ID NO: 308 - DNA, 38 bp, Artificial Sequence
  artificial sequence
gggagagatatcgtctccacccaactgggtcgagtgat

SEQ ID NO: 309 - DNA, 32 bp, Artificial Sequence
  artificial sequence
ctcctgcatcgcaaatacgttgacactgcttt

SEQ ID NO: 310 - DNA, 37 bp, Artificial Sequence
  artificial sequence
ttggttcgcactagtggaagtcactgcatatatactt

SEQ ID NO: 311 - DNA, 47 bp, Artificial Sequence
  artificial sequence
ttccgatgaagcgtacctgggatcgaaagtctccttgccgaagactt

SEQ ID NO: 312 - DNA, 39 bp, Artificial Sequence
  artificial sequence
aaaagttttaaaatctcaagcggtgcgcaaacggcgttt

SEQ ID NO: 313 - DNA, 30 bp, Artificial Sequence
  artificial sequence
ttgcttcttacgtatgcctctaaccgtcat

SEQ ID NO: 314 - DNA, 51 bp, Artificial Sequence
  artificial sequence
cgagcggtgtagcgaacaagccagagcagatgctcggggatccaaatattt

SEQ ID NO: 315 - DNA, 40 bp, Artificial Sequence
  artificial sequence
atcccgcgaaaagatactgcaggacttaaatgcccacttt

SEQ ID NO: 316 - DNA, 32 bp, Artificial Sequence
  artificial sequence
tttaacatgtctagtgtctgttcgtgctatac

SEQ ID NO: 317 - DNA, 51 bp, Artificial Sequence
  artificial sequence
acctaacaatttgagttggatgtccttcggggtgatccgtaggcaccggtt

SEQ ID NO: 318 - DNA, 48 bp, Artificial Sequence
  artificial sequence
ttggaaaacattctgtggcagctttcactagggtcaaaggcaggcgtt

SEQ ID NO: 319 - DNA, 32 bp, Artificial Sequence
  artificial sequence
atggcacccgccgcgcttaatgtttggaacaa

SEQ ID NO: 320 - DNA, 40 bp, Artificial Sequence
  artificial sequence
aactacgatacgggagagtatataataactcgtcggtgta

SEQ ID NO: 321 - DNA, 32 bp, Artificial Sequence
  artificial sequence
gctaaggtcgtgaggcgtcaatagaagctcag

SEQ ID NO: 322 - DNA, 39 bp, Artificial Sequence
  artificial sequence
tttgttaacctaatcaagttttttgggataatggggcga

SEQ ID NO: 323 - DNA, 27 bp, Artificial Sequence
  artificial sequence
gggtcttacaaatgtaaataaacgact

SEQ ID NO: 324 - DNA, 39 bp, Artificial Sequence
  artificial sequence
ccgtctatactccaacgttaaattgggcggagacaaggt

SEQ ID NO: 325 - DNA, 40 bp, Artificial Sequence
  artificial sequence
tacatgcccgcattggattgtccaagccgtatgtgagtcc

SEQ ID NO: 326 - DNA, 24 bp, Artificial Sequence
  artificial sequence
gaccgagttgctcttggaatagtg

SEQ ID NO: 327 - DNA, 32 bp, Artificial Sequence
  artificial sequence
attgcgcccatatgctgaacctacctaggcgg

SEQ ID NO: 328 - DNA, 42 bp, Artificial Sequence
  artificial sequence
agcatcggtaagtacgttgcagcctgcaagatcaccgccttt

SEQ ID NO: 329 - DNA, 48 bp, Artificial Sequence
  artificial sequence
aaccaatacttaccggctgtaggtagtagtagtcgccgtacgtgttcc

SEQ ID NO: 330 - DNA, 31 bp, Artificial Sequence
  artificial sequence
gtatgtggggccagcaaaaggccaggaatat

SEQ ID NO: 331 - DNA, 48 bp, Artificial Sequence
  artificial sequence
aagtctgtggagtctcctttccgtagatgaatctagaagtgctcatca

SEQ ID NO: 332 - DNA, 31 bp, Artificial Sequence
  artificial sequence
cttgcacagtatgctcacgcgggcctcactg

SEQ ID NO: 333 - DNA, 35 bp, Artificial Sequence
  artificial sequence
cccgaaaagtgccacttcggtcagcggaacgtatt

SEQ ID NO: 334 - DNA, 48 bp, Artificial Sequence
  artificial sequence
tggccggtttaacgtattccatagccccctaagagcaaaaggaatagg

SEQ ID NO: 335 - DNA, 40 bp, Artificial Sequence
  artificial sequence
ttgtaagcagctcacgatacctgttgaactcttgcgcata

SEQ ID NO: 336 - DNA, 32 bp, Artificial Sequence
  artificial sequence
tcggccaccattagatggctctcttcggaaaa

SEQ ID NO: 337 - DNA, 40 bp, Artificial Sequence
  artificial sequence
ggcttaccggtctgacagtcccgttagcgcgaccggcgtc

SEQ ID NO: 338 - DNA, 35 bp, Artificial Sequence
  artificial sequence
actaatgcatagggctactcgaggcaagtcgacgc

SEQ ID NO: 339 - DNA, 34 bp, Artificial Sequence
  artificial sequence
ccattgcacgcagtgctatctggccccagtgctg

SEQ ID NO: 340 - DNA, 46 bp, Artificial Sequence
  artificial sequence
gtaaccacattttttgagtccactctcctgttccgaccaccttgac

SEQ ID NO: 341 - DNA, 31 bp, Artificial Sequence
  artificial sequence
ctcgtgcgctattaaagaacgtggcagggcg

SEQ ID NO: 342 - DNA, 47 bp, Artificial Sequence
  artificial sequence
tccccctgggtagaggtggcgaaacccgacaggacccgtaaaaaggc

SEQ ID NO: 343 - DNA, 47 bp, Artificial Sequence
  artificial sequence
cggctcttcttctcagtcttttcaagtgacctaaaagtatctgcgcc

SEQ ID NO: 344 - DNA, 32 bp, Artificial Sequence
  artificial sequence
tcaggaggccggaccactgctacactagaaga

SEQ ID NO: 345 - DNA, 40 bp, Artificial Sequence
  artificial sequence
ttgtcaacttcgacacgaagctccctcccttctttgttaa

SEQ ID NO: 346 - DNA, 33 bp, Artificial Sequence
  artificial sequence
aaatagggctgtcatacaaacgatcatacaggc

SEQ ID NO: 347 - DNA, 32 bp, Artificial Sequence
  artificial sequence
agtaaattatggtcctgggcacagcaattttt

SEQ ID NO: 348 - DNA, 48 bp, Artificial Sequence
  artificial sequence
ggaagcgcgcacggcggctccgcccgcgttgctggcgtttatataaca

SEQ ID NO: 349 - DNA, 45 bp, Artificial Sequence
  artificial sequence
tttctcatgttaatatatcagctccacccactacgtgaaccgttc

SEQ ID NO: 350 - DNA, 32 bp, Artificial Sequence
  artificial sequence
ggtcgttcgaagtggtgaagattacaccaggc

SEQ ID NO: 351 - DNA, 48 bp, Artificial Sequence
  artificial sequence
ggtacggatttcctagacaaaaatattcctaaaaagatacggtcaatg

SEQ ID NO: 352 - DNA, 31 bp, Artificial Sequence
  artificial sequence
aacattctgacccggcgtcaacaccagcgtt

SEQ ID NO: 353 - DNA, 48 bp, Artificial Sequence
  artificial sequence
ctcccacatttcccatcagtcagcatctcagtcaggaaagactaaccg

SEQ ID NO: 354 - DNA, 40 bp, Artificial Sequence
  artificial sequence
cgacgctcaagtcggtgaccagggtatcaccacgtggcgc

SEQ ID NO: 355 - DNA, 40 bp, Artificial Sequence
  artificial sequence
attttgtaggatccaccgaccttcaccttcgtcagtattt

SEQ ID NO: 356 - DNA, 45 bp, Artificial Sequence
  artificial sequence
atttcacaattcgcctaatcgagaataaagacggaaggaaagttg

SEQ ID NO: 357 - DNA, 32 bp, Artificial Sequence
  artificial sequence
cggacgcagcccagcaggagctggagtagtca

SEQ ID NO: 358 - DNA, 40 bp, Artificial Sequence
  artificial sequence
tgagtaaattttaaatcaatctaaaggatccgggcctaac

SEQ ID NO: 359 - DNA, 23 bp, Artificial Sequence
  artificial sequence
aaccataccgctacgtaaaaagt

SEQ ID NO: 360 - DNA, 33 bp, Artificial Sequence
  artificial sequence
tttaacgaccgggcaatagaactttagtaattt

SEQ ID NO: 361 - DNA, 42 bp, Artificial Sequence
  artificial sequence
aggagttagcgtgaagcacatcgtactagcctgcgacccttt

SEQ ID NO: 362 - DNA, 45 bp, Artificial Sequence
  artificial sequence
taagtagataactttgcaccagccctgaaaggactgtcgttaatt

SEQ ID NO: 363 - DNA, 36 bp, Artificial Sequence
  artificial sequence
ttgtatgagctctgggtctgaggtctcaaggttgac

SEQ ID NO: 364 - DNA, 37 bp, Artificial Sequence
  artificial sequence
ttttatcagaattcagctcttctagcctgggggttaa

SEQ ID NO: 365 - DNA, 37 bp, Artificial Sequence
  artificial sequence
atcttggtcattgctaaggaagcataacacatggatt

SEQ ID NO: 366 - DNA, 52 bp, Artificial Sequence
  artificial sequence
aaactctcaaggatttttcttaagcatttttcttttacttttacggggtcga

SEQ ID NO: 367 - DNA, 48 bp, Artificial Sequence
  artificial sequence
ccaggcagcggaaccccagacatttttgggctggaagccgaggcccaa

SEQ ID NO: 368 - DNA, 47 bp, Artificial Sequence
  artificial sequence
gttgagtgttgttccagttcgctagctttttttagagcgcaaaatag

SEQ ID NO: 369 - DNA, 44 bp, Artificial Sequence
  artificial sequence
gcaagtgtttttagcggtcacgctgcgcggtgccgtatgctaaa

SEQ ID NO: 370 - DNA, 44 bp, Artificial Sequence
  artificial sequence
tacggccgggccgaaacgtattgaaaagcacttttttaatcgga

SEQ ID NO: 371 - DNA, 44 bp, Artificial Sequence
  artificial sequence
tctggtgagtttttactcaaccaagtttctcttagttccgcgca

SEQ ID NO: 372 - DNA, 28 bp, Artificial Sequence
  artificial sequence
gttcttgctccatttttgctggcaacta

SEQ ID NO: 373 - DNA, 48 bp, Artificial Sequence
  artificial sequence
acgctgatgactcggcaaaatctttttcttataaatcaccgagatagg

SEQ ID NO: 374 - DNA, 38 bp, Artificial Sequence
  artificial sequence
cactttgcctcgggatgggattgcctttttttgtgcca

SEQ ID NO: 375 - DNA, 41 bp, Artificial Sequence
  artificial sequence
cattgcgaccctaaagaatgtatttagaatttttaataaac

SEQ ID NO: 376 - DNA, 30 bp, Artificial Sequence
  artificial sequence
acagtatttggtatttttttgcgctacaga

SEQ ID NO: 377 - DNA, 38 bp, Artificial Sequence
  artificial sequence
aaatgaagcttggtctgacagttactttttaatgctta

SEQ ID NO: 378 - DNA, 38 bp, Artificial Sequence
  artificial sequence
agtatagggaccagtgacggtaattttttgaatgagcg

SEQ ID NO: 379 - DNA, 38 bp, Artificial Sequence
  artificial sequence
tcaggcggtcttcacctagatccttttttttaaattaa

SEQ ID NO: 380 - DNA, 47 bp, Artificial Sequence
  artificial sequence
tagcacatgccatccgtttttaagatgcttattgaagccgatggatt

SEQ ID NO: 381 - DNA, 30 bp, Artificial Sequence
  artificial sequence
tccataagacactttttggagggaacctgc

SEQ ID NO: 382 - DNA, 46 bp, Artificial Sequence
  artificial sequence
atcagtgacatccatagttgcctgtttttctccccgtcgtgtagat

SEQ ID NO: 383 - DNA, 48 bp, Artificial Sequence
  artificial sequence
ttatacagaataacgagtcattttcggtccaactcaagcaggttctgg

SEQ ID NO: 384 - DNA, 48 bp, Artificial Sequence
  artificial sequence
ataaataagttgcctgacatttttttcgaataacttgcagaccttgga

SEQ ID NO: 385 - DNA, 40 bp, Artificial Sequence
  artificial sequence
aagaattacgtttttgtaaatgccatttttgatgggcagc

SEQ ID NO: 386 - DNA, 40 bp, Artificial Sequence
  artificial sequence
gtttgtgcgttttttatcattaagctttttggcgtccaaa

SEQ ID NO: 387 - DNA, 56 bp, Artificial Sequence
  artificial sequence
ctggcgtttttggtaattgcgggctgatcttttttgattgctagtcatggtcttgg

SEQ ID NO: 388 - DNA, 52 bp, Artificial Sequence
  artificial sequence
actgttcctacgcagttttttgcaatctgactgctggccgtttttccggagt

SEQ ID NO: 389 - DNA, 48 bp, Artificial Sequence
  artificial sequence
agcaatacgggaggcacacacgcttttttacgacggataggcgaaggc

SEQ ID NO: 390 - DNA, 48 bp, Artificial Sequence
  artificial sequence
ggcgtttcagacgaatttttcagggtcctttttctgctgtagtaactt

SEQ ID NO: 391 - DNA, 33 bp, Artificial Sequence
  artificial sequence
ggtcctatcgcttcgaacgttttttattacgca

SEQ ID NO: 392 - DNA, 86 bp, Artificial Sequence
  artificial sequence
tacatagttcattgtcgggcagttaatcctttttgcaaatagagttacgtcgtttttaattatccttttgcaatgcagggattctt

SEQ ID NO: 393 - DNA, 36 bp, Artificial Sequence
  artificial sequence
tactcaagatttttctcataggtttttgattcggtg

SEQ ID NO: 394 - DNA, 36 bp, Artificial Sequence
  artificial sequence
agtgtcctgtttttcggaaccttttttattgtctat

SEQ ID NO: 395 - DNA, 77 bp, Artificial Sequence
  artificial sequence
atccgcgtccatgtccacgaatatttttccctatcgtttttgtgactaatccggggccgggccgctctgcgtgtacg

SEQ ID NO: 396 - DNA, 44 bp, Artificial Sequence
  artificial sequence
gacgcccgaatttttactgggctagagcctctttggtcttcata

SEQ ID NO: 397 - DNA, 46 bp, Artificial Sequence
  artificial sequence
tgttggcatagagtacatcaaacaattttttaagaaaccgtagaac

SEQ ID NO: 398 - DNA, 56 bp, Artificial Sequence
  artificial sequence
cacttacgcctgagagagatttttctgtattctgttagttgtcatacataggttgt

SEQ ID NO: 399 - DNA, 42 bp, Artificial Sequence
  artificial sequence
gctttatacaactctcgataagacgttagcatcttactctga

SEQ ID NO: 400 - DNA, 37 bp, Artificial Sequence
  artificial sequence
tctcagtcataactgccataataaccaagtgtcgtac

SEQ ID NO: 401 - DNA, 48 bp, Artificial Sequence
  artificial sequence
cttgaacgcctggctttttatcgggggtctttttagcgaattctatac

SEQ ID NO: 402 - DNA, 40 bp, Artificial Sequence
  artificial sequence
acaaacccccatttttgttcatagtttttaggcattgttc

SEQ ID NO: 403 - DNA, 44 bp, Artificial Sequence
  artificial sequence
tgcgagccgcgttttaacattgtagcagcctctttttaggataa

SEQ ID NO: 404 - DNA, 58 bp, Artificial Sequence
  artificial sequence
ctaggtgcgaggtttttattatatcgcacgtttgaatggcctcttttttgtcgtcgtg

SEQ ID NO: 405 - DNA, 36 bp, Artificial Sequence
  artificial sequence
cccgcagactttttaagcagtctttttccgggtgct

SEQ ID NO: 406 - DNA, 39 bp, Artificial Sequence
  artificial sequence
ttttgtaatgtgtgacatagcgaatcccacctcgtttcg

SEQ ID NO: 407 - DNA, 48 bp, Artificial Sequence
  artificial sequence
aatccgcctcgggagatcttttttaaaggactgaaataatcctcacag

SEQ ID NO: 408 - DNA, 36 bp, Artificial Sequence
  artificial sequence
tcaagattgttttttgatttggttttttacgctaag

SEQ ID NO: 409 - DNA, 43 bp, Artificial Sequence
  artificial sequence
gcgaatagacctgatcttgagcgcggaatcttcgggctgttaa

SEQ ID NO: 410 - DNA, 44 bp, Artificial Sequence
  artificial sequence
ctaagttttggctgcggattggtttttgcagaaggtcaagcgca

SEQ ID NO: 411 - DNA, 64 bp, Artificial Sequence
  artificial sequence
caatcgttttttgaacgttcgttttttcagtggttgccgttataagtcattcgtcgggagcgcg

SEQ ID NO: 412 - DNA, 44 bp, Artificial Sequence
  artificial sequence
gaacttctactcgcgatgcaaatttttttaagtcacgtcgctaa

SEQ ID NO: 413 - DNA, 40 bp, Artificial Sequence
  artificial sequence
tcaaagtatcgtttttaaagaatttttttgcccaaccagc

SEQ ID NO: 414 - DNA, 40 bp, Artificial Sequence
  artificial sequence
ggctacatagtacgcattccatcctgcagacaagggacac

SEQ ID NO: 415 - DNA, 47 bp, Artificial Sequence
  artificial sequence
tcggtgtacgaaagagcgagaagtcgaccttttttgtttatatgggg

SEQ ID NO: 416 - DNA, 32 bp, Artificial Sequence
  artificial sequence
cgaaaacggtctctaagaatgacatcggacga

SEQ ID NO: 417 - DNA, 41 bp, Artificial Sequence
  artificial sequence
ggttaccactaaggtcaaatacaagaatgtgcctacgcgaa

SEQ ID NO: 418 - DNA, 47 bp, Artificial Sequence
  artificial sequence
ggatcgcttccgaccaccctggatgagctcatgggactttacggtga

SEQ ID NO: 419 - DNA, 28 bp, Artificial Sequence
  artificial sequence
gtgtttccaacgaccactggagggtagc

SEQ ID NO: 420 - DNA, 29 bp, Artificial Sequence
  artificial sequence
caaaattaatcatcctccccttggtgcat

SEQ ID NO: 421 - DNA, 29 bp, Artificial Sequence
  artificial sequence
cctcgcttatgttggctcctccaagaggt

SEQ ID NO: 422 - DNA, 27 bp, Artificial Sequence
  artificial sequence
tagccacgtgtagtataccaggattaa

SEQ ID NO: 423 - DNA, 29 bp, Artificial Sequence
  artificial sequence
cccggacaagctgaccagggggtatgatg

SEQ ID NO: 424 - DNA, 28 bp, Artificial Sequence
  artificial sequence
tgttaagacgtatagatctaggtcgccc

SEQ ID NO: 425 - DNA, 70 bp, Artificial Sequence
  artificial sequence
ggtaactatcagtggacgaatccacttgcctgaaactagaatgccacctgactattctatgagggggata

SEQ ID NO: 426 - DNA, 80 bp, Artificial Sequence
  artificial sequence
agaaagcgagagcttgtagccccacagaactttgactatatccctaacatgcagctaaaccgactcggctcaatcacagg

SEQ ID NO: 427 - DNA, 23 bp, Artificial Sequence
  artificial sequence
agaggacgggcgaaattttaaat

SEQ ID NO: 428 - DNA, 24 bp, Artificial Sequence
  artificial sequence
agcgtaaacctccgtgcagaacac

SEQ ID NO: 429 - DNA, 30 bp, Artificial Sequence
  artificial sequence
atacattaataattggtctctcgtgagcaa

SEQ ID NO: 430 - DNA, 32 bp, Artificial Sequence
  artificial sequence
ttttctactcgtacctctaattaaacgtcgtc

SEQ ID NO: 431 - DNA, 46 bp, Artificial Sequence
  artificial sequence
tgctatggtctcacggaagccgtacttcctgaaaatctccagacga

SEQ ID NO: 432 - DNA, 16 bp, Artificial Sequence
  artificial sequence
aatatcttgaggtaag

SEQ ID NO: 433 - DNA, 31 bp, Artificial Sequence
  artificial sequence
gcagagagccacagatcctcgtgaccactcg

SEQ ID NO: 434 - DNA, 26 bp, Artificial Sequence
  artificial sequence
actaatagcgttaatcatcgttcagt

SEQ ID NO: 435 - DNA, 33 bp, Artificial Sequence
  artificial sequence
gcgcctgcgttctgcgttctcatcggtaccaag

SEQ ID NO: 436 - DNA, 27 bp, Artificial Sequence
  artificial sequence
gacgttatgtgattagagtgactattc

SEQ ID NO: 437 - DNA, 73 bp, Artificial Sequence
  artificial sequence
agcgttgtcgtcctacatcgaatccacttgcctgaaactagaatgccacctgactatcgtaactacttggcat

SEQ ID NO: 438 - DNA, 64 bp, Artificial Sequence
  artificial sequence
ttggtacaaccgaatcagaactttgactatatccctaacatgcagctaaaccgagcggccattc

SEQ ID NO: 439 - DNA, 39 bp, Artificial Sequence
  artificial sequence
aaaagcggtgttgccatagtttgtgaatccgcctccatc

SEQ ID NO: 440 - DNA, 19 bp, Artificial Sequence
  artificial sequence
tggtgtcacgggcagcact

SEQ ID NO: 441 - DNA, 40 bp, Artificial Sequence
  artificial sequence
caacgatcaaggcagtgttatcactcagaagtatgtgcaa

SEQ ID NO: 442 - DNA, 39 bp, Artificial Sequence
  artificial sequence
gtcctccgatcgttgtcatggttatctcgtcgtttggta

SEQ ID NO: 443 - DNA, 18 bp, Artificial Sequence
  artificial sequence
gataccgcgcgcaacgtt

SEQ ID NO: 444 - DNA, 36 bp, Artificial Sequence
  artificial sequence
gctcaccggctccaggaagtggtagagtaaggaagg

SEQ ID NO: 445 - DNA, 32 bp, Artificial Sequence
  artificial sequence
gccagttagggaagctcctgcaactttcccac

SEQ ID NO: 446 - DNA, 47 bp, Artificial Sequence
  artificial sequence
accagccagccgtagttctggcttcacccatgtagttggccgcgagt

SEQ ID NO: 447 - DNA, 20 bp, Artificial Sequence
  artificial sequence
gtctattaatttagctcctt

SEQ ID NO: 448 - DNA, 75 bp, Artificial Sequence
  artificial sequence
cccctgacgagcatcagatccgaatccacttgcctgaaactagaatgccacctgactatgcgcaatttatcagca

SEQ ID NO: 449 - DNA, 76 bp, Artificial Sequence
  artificial sequence
atgggaggaagctccttgtaccagaactttgactatatccctaacatgcagctaaaccgagatccttcagctccgg

SEQ ID NO: 450 - DNA, 39 bp, Artificial Sequence
  artificial sequence
atagtcaggtggcattctagtttcaggcaagtggattcg

SEQ ID NO: 451 - DNA, 39 bp, Artificial Sequence
  artificial sequence
tcggtttagctgcatgttagggatatagtcaaagttctg

SEQ ID NO: 452 - DNA, 36 bp, Artificial Sequence
  artificial sequence
atcagtgacatccatagttgcctgattatacatcta

SEQ ID NO: 453 - DNA, 58 bp, Artificial Sequence
  artificial sequence
tagcacatgccatccgtttttaagatgcttattgaagccgatggattttatacatcta

SEQ ID NO: 454 - DNA, 35 bp, Artificial Sequence
  artificial sequence
tccataagacactttttggagggattatacatcta

SEQ ID NO: 455 - DNA, 57 bp, Artificial Sequence
  artificial sequence
ctccccgtcgtgtagataactacgatacgggagagtatataataactcgtcggtgta

SEQ ID NO: 456 - DNA, 37 bp, Artificial Sequence
  artificial sequence
tgttggcatagagtacatcaaacaatttatacatcta

SEQ ID NO: 457 - DNA, 38 bp, Artificial Sequence
  artificial sequence
taagaaaccgtagaacgacgcccgaacttatacatcta

SEQ ID NO: 458 - DNA, 48 bp, Artificial Sequence
  artificial sequence
atccgcgtccatgtccacgaatatttttccctatcgtttatacatcta

SEQ ID NO: 459 - DNA, 29 bp, Artificial Sequence
  artificial sequence
actgggctagagcctctttggtcttcata

SEQ ID NO: 460 - DNA, 36 bp, Artificial Sequence
  artificial sequence
gtgactaatccggggccgggccgctctgcgtgtacg

SEQ ID NO: 461 - DNA, 42 bp, Artificial Sequence
  artificial sequence
tcggtgtacgaaagagcgagaagtcgacctgttatacatcta

SEQ ID NO: 462 - DNA, 51 bp, Artificial Sequence
  artificial sequence
ggctacatagtacgcattccatcctgcagacaagggacacttatacatcta

SEQ ID NO: 463 - DNA, 47 bp, Artificial Sequence
  artificial sequence
gcccaaccagctcaaagtatcgtttttaaagaatttttatacatcta

SEQ ID NO: 464 - DNA, 49 bp, Artificial Sequence
  artificial sequence
gtttatatggggggcctggacaactggccgagggctgtgtccaggtgct

SEQ ID NO: 465 - DNA, 10 bp, Artificial Sequence
  artificial sequence
ctagatgtat

SEQ ID NO: 466 - DNA, 49 bp, Artificial Sequence
  artificial sequence
cgaaacgggataactcccagtcacgacggtgctgccgcaacttctggtg

SEQ ID NO: 467 - DNA, 49 bp, Artificial Sequence
  artificial sequence
gaattataaaagggcatatggtttaccaatacatagtatgttaacaaag

SEQ ID NO: 468 - DNA, 42 bp, Artificial Sequence
  artificial sequence
caccgattattttcacgacttgcgggagccaaagaccaccgt

SEQ ID NO: 469 - DNA, 35 bp, Artificial Sequence
  artificial sequence
gagatagctcatttgccgcagctttcagcccggaa

SEQ ID NO: 470 - DNA, 42 bp, Artificial Sequence
  artificial sequence
tagctcttaagtcctgaacaattttttcgtaaagtcgcactc

SEQ ID NO: 471 - DNA, 42 bp, Artificial Sequence
  artificial sequence
tacagcgaatcggctgtctttcaggctgaaggcgatgtgagc

SEQ ID NO: 472 - DNA, 28 bp, Artificial Sequence
  artificial sequence
ccgtggtgaagggacggatcaacataaa

SEQ ID NO: 473 - DNA, 49 bp, Artificial Sequence
  artificial sequence
tgaatatgctttgatattcatttcaattcatttaaacagtacaattaat

SEQ ID NO: 474 - DNA, 49 bp, Artificial Sequence
  artificial sequence
ttgcgtatttccagatgagtgagctaacgctcacattcgtaaacgcgtg

SEQ ID NO: 475 - DNA, 42 bp, Artificial Sequence
  artificial sequence
ggtttttcccgttgcgctcactgcccgcttgggcgtacttct

SEQ ID NO: 476 - DNA, 49 bp, Artificial Sequence
  artificial sequence
cacggaaaaataagagaatatcgcctgtttatcaaagcctccggcggcc

SEQ ID NO: 477 - DNA, 35 bp, Artificial Sequence
  artificial sequence
ctaccatttgaggaggaagcaaacggcatcagatg

SEQ ID NO: 478 - DNA, 42 bp, Artificial Sequence
  artificial sequence
ttaaacgaacggagatttgtataattgtcaaatcaatacata

SEQ ID NO: 479 - DNA, 49 bp, Artificial Sequence
  artificial sequence
cgacaaataggcagggcttaattgagaacaaattcatcataaccgaccg

SEQ ID NO: 480 - DNA, 56 bp, Artificial Sequence
  artificial sequence
caccaccctattagcaaaattttagcgtcagactggtgtctggtttagcaatcccc

SEQ ID NO: 481 - DNA, 49 bp, Artificial Sequence
  artificial sequence
ctttgagtgccactaccaagcgcgaaacttgctttcgatatatacgagg

SEQ ID NO: 482 - DNA, 35 bp, Artificial Sequence
  artificial sequence
gagttgcgcgaaaagactccaacgtcaacactacg

SEQ ID NO: 483 - DNA, 49 bp, Artificial Sequence
  artificial sequence
cgccgccccaccctatagcccccttatttgaaacataataagggatagc

SEQ ID NO: 484 - DNA, 35 bp, Artificial Sequence
  artificial sequence
accaccaaccgttccagtaagcgtcatagagccgc

SEQ ID NO: 485 - DNA, 49 bp, Artificial Sequence
  artificial sequence
caccagatcagagcttttcatcggcattggctgaggatgataaatcgtc

SEQ ID NO: 486 - DNA, 44 bp, Artificial Sequence
  artificial sequence
gcaaagacattttcatttggggcataacctgaagtttatatgca

SEQ ID NO: 487 - DNA, 54 bp, Artificial Sequence
  artificial sequence
gcattaacatcccagagcagcgacagaatcaagtataacattcgcaaacagttc

SEQ ID NO: 488 - DNA, 42 bp, Artificial Sequence
  artificial sequence
tttagaaatgtgtaggtaaagaaatcacaaattaaacaaagg

SEQ ID NO: 489 - DNA, 49 bp, Artificial Sequence
  artificial sequence
agagccgagcattggaaagcgcagtctcgtactggtgaaagttcagtac

SEQ ID NO: 490 - DNA, 42 bp, Artificial Sequence
  artificial sequence
tcagggacgacaataaaaagcctgttaccttgaaaactggtt

SEQ ID NO: 491 - DNA, 42 bp, Artificial Sequence
  artificial sequence
atccggacaattttaacgccagggtttctcaccggaaggctt

SEQ ID NO: 492 - DNA, 49 bp, Artificial Sequence
  artificial sequence
atttctgactttctaatatcccatcctattttccggcaaacgtagaacg

SEQ ID NO: 493 - DNA, 42 bp, Artificial Sequence
  artificial sequence
gccagtaagaaagccgcagctcaacagtagaggcattttcga

SEQ ID NO: 494 - DNA, 28 bp, Artificial Sequence
  artificial sequence
gccaacatgtaattaggtaaaatgttca

SEQ ID NO: 495 - DNA, 28 bp, Artificial Sequence
  artificial sequence
ataccaagttacaaactttaacgtcaga

SEQ ID NO: 496 - DNA, 42 bp, Artificial Sequence
  artificial sequence
aataaccaaaagaagatgatgaaacaactgcattaaagaaac

SEQ ID NO: 497 - DNA, 35 bp, Artificial Sequence
  artificial sequence
gtgccaggtgtaaagcctgggacgagcctccccgg

SEQ ID NO: 498 - DNA, 42 bp, Artificial Sequence
  artificial sequence
gactttttcatgaggaagtaatattcattaggcttgcaggga

SEQ ID NO: 499 - DNA, 42 bp, Artificial Sequence
  artificial sequence
ttaggagcactaacaactatgaaaaccgtctaaagcatcacc

SEQ ID NO: 500 - DNA, 49 bp, Artificial Sequence
  artificial sequence
cacgtaaaatatataacaaaatggtgtgttcagcagactaccatttatc

SEQ ID NO: 501 - DNA, 35 bp, Artificial Sequence
  artificial sequence
tatctaaacatttgttaaaagtttgagtaacatcg

SEQ ID NO: 502 - DNA, 49 bp, Artificial Sequence
  artificial sequence
gaataatgctcgaaattccacacctgcagccagcggcagtgttttcacg

SEQ ID NO: 503 - DNA, 35 bp, Artificial Sequence
  artificial sequence
aattgcgaatggaacaatttccgtcataaacatcc

SEQ ID NO: 504 - DNA, 49 bp, Artificial Sequence
  artificial sequence
tgacaagaaagctgttaaaaggagcctttcatcgcagggaaccgttcca

SEQ ID NO: 505 - DNA, 35 bp, Artificial Sequence
  artificial sequence
aaccggactgaccaactttgaaatcatactgataa

SEQ ID NO: 506 - DNA, 45 bp, Artificial Sequence
  artificial sequence
gcggaactgcgcgatcagggcgaagaactcaaacttgaggaggcc

SEQ ID NO: 507 - DNA, 35 bp, Artificial Sequence
  artificial sequence
ccctcagatgacaacttgataaaaggaacaactaa

SEQ ID NO: 508 - DNA, 35 bp, Artificial Sequence
  artificial sequence
agcatgtagaaaccagggcgaggcgaaacggattc

SEQ ID NO: 509 - DNA, 35 bp, Artificial Sequence
  artificial sequence
aatcaatccatgtttaccagtaggtggaacgacgg

SEQ ID NO: 510 - DNA, 35 bp, Artificial Sequence
  artificial sequence
gaacgggaataagactgaatcccagctttcatcaa

SEQ ID NO: 511 - DNA, 42 bp, Artificial Sequence
  artificial sequence
ttaaagcggggtcaggaacctccgtcgagagggttccaaagc

SEQ ID NO: 512 - DNA, 28 bp, Artificial Sequence
  artificial sequence
cagaatgacaggaggttgagggaaccgc

SEQ ID NO: 513 - DNA, 49 bp, Artificial Sequence
  artificial sequence
tggcatcgatacatgttgattctgtagctcaacattttgcggctattat

SEQ ID NO: 514 - DNA, 45 bp, Artificial Sequence
  artificial sequence
actaatatgcaatgctcagatttagtttgaccataaatggaagat

SEQ ID NO: 515 - DNA, 42 bp, Artificial Sequence
  artificial sequence
ttatttagggaaggttttatttcaacgagggtgagaataagt

SEQ ID NO: 516 - DNA, 35 bp, Artificial Sequence
  artificial sequence
atcaatataaaagaattaagaccgaggaaacgcaa

SEQ ID NO: 517 - DNA, 35 bp, Artificial Sequence
  artificial sequence
gaaaattcgacattcaaccgatattcatgcaaaat

SEQ ID NO: 518 - DNA, 49 bp, Artificial Sequence
  artificial sequence
ccagcagagcaagcccaccagaaggagcgtggcgatgaaccaataacat

SEQ ID NO: 519 - DNA, 35 bp, Artificial Sequence
  artificial sequence
gttgctattttgcacgctaactttatccgtcaaaa

SEQ ID NO: 520 - DNA, 49 bp, Artificial Sequence
  artificial sequence
ccagtgcgccagcttcggtgcagccagctttccggtcaggaaaccgtaa

SEQ ID NO: 521 - DNA, 28 bp, Artificial Sequence
  artificial sequence
ggttgtgtgctgattgccgcgcggggtc

SEQ ID NO: 522 - DNA, 42 bp, Artificial Sequence
  artificial sequence
aaaatccatgaagggtctcgttaacggaacgtgccatgccaa

SEQ ID NO: 523 - DNA, 35 bp, Artificial Sequence
  artificial sequence
atttatcgcgcagatttagtatcatatgatgggta

SEQ ID NO: 524 - DNA, 35 bp, Artificial Sequence
  artificial sequence
acctgagggattcgcctgattacagtaaataaaga

SEQ ID NO: 525 - DNA, 43 bp, Artificial Sequence
  artificial sequence
aattgcgagataggggctgtgtgaaatttgccccctgagagtc

SEQ ID NO: 526 - DNA, 35 bp, Artificial Sequence
  artificial sequence
tattaaaaatcaaggaaagccgcgctggcaagtgt

SEQ ID NO: 527 - DNA, 42 bp, Artificial Sequence
  artificial sequence
atcaataccagtgagacgggcccttatagttgttccagtttg

SEQ ID NO: 528 - DNA, 35 bp, Artificial Sequence
  artificial sequence
gatgatggcaattcgggagcctaaagcatcacgca

SEQ ID NO: 529 - DNA, 28 bp, Artificial Sequence
  artificial sequence
catcgagaatcattaccgcgcgaggcgt

SEQ ID NO: 530 - DNA, 45 bp, Artificial Sequence
  artificial sequence
aagccgtgtcagttacaaaatctttacagagagaataacacgagc

SEQ ID NO: 531 - DNA, 42 bp, Artificial Sequence
  artificial sequence
caccagttggcatgaacgcaatcgcattaaattttgagcaag

SEQ ID NO: 532 - DNA, 21 bp, Artificial Sequence
  artificial sequence
acggaaagcacccaaaagaac

SEQ ID NO: 533 - DNA, 42 bp, Artificial Sequence
  artificial sequence
tttccagaagattatttagcgaacctcctcgtaggaacaagc

SEQ ID NO: 534 - DNA, 35 bp, Artificial Sequence
  artificial sequence
agcaccaatattgacggaaatttgagggtgtcaca

SEQ ID NO: 535 - DNA, 28 bp, Artificial Sequence
  artificial sequence
tttagtgcgtaaaaagacgcagaaacag

SEQ ID NO: 536 - DNA, 49 bp, Artificial Sequence
  artificial sequence
gctaatgcaccggattaccagactgttgccctgcgtccaatctcttctg

SEQ ID NO: 537 - DNA, 40 bp, Artificial Sequence
  artificial sequence
aagaagtgagtgaataaagatcaaaaaatcggccaacgcg

SEQ ID NO: 538 - DNA, 35 bp, Artificial Sequence
  artificial sequence
tcatcatattcctgtgacgggttttttggcaatac

SEQ ID NO: 539 - DNA, 42 bp, Artificial Sequence
  artificial sequence
ggtgccgcccgattacgctgcgcgtaacagggcgcagtgagg

SEQ ID NO: 540 - DNA, 35 bp, Artificial Sequence
  artificial sequence
gggtcgagaacaagaaatcggcaaaatcaacagct

SEQ ID NO: 541 - DNA, 35 bp, Artificial Sequence
  artificial sequence
tcacccagaacgtgtcctgtttgatggtgcctggc

SEQ ID NO: 542 - DNA, 49 bp, Artificial Sequence
  artificial sequence
aaatctaactgataatggctattagtctcgggagctaaacgcagattca

SEQ ID NO: 543 - DNA, 28 bp, Artificial Sequence
  artificial sequence
cagcagcttgctggtaatatctctgaaa

SEQ ID NO: 544 - DNA, 42 bp, Artificial Sequence
  artificial sequence
aatatctttgctgaacctcaatgagagcccattaatggcaca

SEQ ID NO: 545 - DNA, 49 bp, Artificial Sequence
  artificial sequence
gccgcttgcataaccgaggtggcgaataataatttaacgatcctacaac

SEQ ID NO: 546 - DNA, 42 bp, Artificial Sequence
  artificial sequence
ttgagatcgaaatcaggcgcagacggtcaagaggagtaatct

SEQ ID NO: 547 - DNA, 42 bp, Artificial Sequence
  artificial sequence
aatttctcgattatacgaaggcaccaacaacggctatcgtca

SEQ ID NO: 548 - DNA, 44 bp, Artificial Sequence
  artificial sequence
tagcaaggagggtaggccggaacgttaatattttgcacaatcat

SEQ ID NO: 549 - DNA, 35 bp, Artificial Sequence
  artificial sequence
taatcctgattgttcatagctgtttcaacccgccg

SEQ ID NO: 550 - DNA, 42 bp, Artificial Sequence
  artificial sequence
cattccatttgcctaagcaataaagcctaataaatgaaaagg

SEQ ID NO: 551 - DNA, 46 bp, Artificial Sequence
  artificial sequence
aaacttcttgagccatttgggaattttacgcaaaggtggtcagctc

SEQ ID NO: 552 - DNA, 42 bp, Artificial Sequence
  artificial sequence
ataaatcaacagaacagtaccttttacatcgggtgttatttg

SEQ ID NO: 553 - DNA, 42 bp, Artificial Sequence
  artificial sequence
tagagctattatcagattgcccttcaccggttccgagtccac

SEQ ID NO: 554 - DNA, 49 bp, Artificial Sequence
  artificial sequence
gaaaggaagggaaaaaagaaaggtccacgcatagattagagctcatttt

SEQ ID NO: 555 - DNA, 37 bp, Artificial Sequence
  artificial sequence
caccgtactgcgaacgagtaacctgagagtctgaata

SEQ ID NO: 556 - DNA, 28 bp, Artificial Sequence
  artificial sequence
ttaaatcagcctaatttgcagaggaacg

SEQ ID NO: 557 - DNA, 42 bp, Artificial Sequence
  artificial sequence
tctccaatacagccctcatagttagcgttttcacgtatcagc

SEQ ID NO: 558 - DNA, 49 bp, Artificial Sequence
  artificial sequence
tcaccgtaccaactttcaacagtttcagcggagtgaattttcgaaccca

SEQ ID NO: 559 - DNA, 42 bp, Artificial Sequence
  artificial sequence
caggcgggcaaactaaatatcgcgttttttagactttttaac

SEQ ID NO: 560 - DNA, 28 bp, Artificial Sequence
  artificial sequence
ttaggattagcgggttagagaagaggaa

SEQ ID NO: 561 - DNA, 28 bp, Artificial Sequence
  artificial sequence
actaaagtccttttcggattgcatcaaa

SEQ ID NO: 562 - DNA, 42 bp, Artificial Sequence
  artificial sequence
taatgcccaattatcagtataaagctaaatcggaaagtagta

SEQ ID NO: 563 - DNA, 42 bp, Artificial Sequence
  artificial sequence
ctatcagaatcgatcagaaaagccccaaaaacacaggagcaa

SEQ ID NO: 564 - DNA, 49 bp, Artificial Sequence
  artificial sequence
gagatcttgccggagccggaatacttttgcgggagaagccaattaccat

SEQ ID NO: 565 - DNA, 42 bp, Artificial Sequence
  artificial sequence
ggaattatttttgaaaactagcatgtatagctatctaataac

SEQ ID NO: 566 - DNA, 42 bp, Artificial Sequence
  artificial sequence
ttaccagaaagtaaaagcccaataataatgttaaacaacata

SEQ ID NO: 567 - DNA, 35 bp, Artificial Sequence
  artificial sequence
atgaaaagagaattttgagcgctaatataaataat

SEQ ID NO: 568 - DNA, 42 bp, Artificial Sequence
  artificial sequence
ccggaaagggacgattggtgtagatgggcattaaattaagtt

SEQ ID NO: 569 - DNA, 35 bp, Artificial Sequence
  artificial sequence
tcagcgtggtgcccgggcctcatttacgtttgtga

SEQ ID NO: 570 - DNA, 42 bp, Artificial Sequence
  artificial sequence
tgtgataaatttcagcaagacaaagaacccgggtctataaag

SEQ ID NO: 571 - DNA, 42 bp, Artificial Sequence
  artificial sequence
tgaaatattactagaaacaacgtaattctgtccagaaacaac

SEQ ID NO: 572 - DNA, 21 bp, Artificial Sequence
  artificial sequence
tagaatcctttttttagattt

SEQ ID NO: 573 - DNA, 49 bp, Artificial Sequence
  artificial sequence
tttccctttaagactgggttatataactctttgctatttgaaggcgaat

SEQ ID NO: 574 - DNA, 28 bp, Artificial Sequence
  artificial sequence
ccgtgagcctcctctagctgcggccaga

SEQ ID NO: 575 - DNA, 35 bp, Artificial Sequence
  artificial sequence
cctgttcgggccgtcactgcgcgcctgtccgggtt

SEQ ID NO: 576 - DNA, 35 bp, Artificial Sequence
  artificial sequence
cggtttctgccagctcatggttggattaccagggt

SEQ ID NO: 577 - DNA, 35 bp, Artificial Sequence
  artificial sequence
gagcgggctttcctcaggaacggtacgcattagta

SEQ ID NO: 578 - DNA, 35 bp, Artificial Sequence
  artificial sequence
tttttgagccctaaaacattacgtcaatagataat

SEQ ID NO: 579 - DNA, 42 bp, Artificial Sequence
  artificial sequence
gacaataccagtcatggattatttacatatcggccaaatgaa

SEQ ID NO: 580 - DNA, 35 bp, Artificial Sequence
  artificial sequence
gccatcttttcatactatttcgtgcctttaatagt

SEQ ID NO: 581 - DNA, 35 bp, Artificial Sequence
  artificial sequence
tattaaacaagcaaatcagatatagaaaattccaa

SEQ ID NO: 582 - DNA, 42 bp, Artificial Sequence
  artificial sequence
aaaaatcaaaaaaggctcctcaactttaaggacgttaacgga

SEQ ID NO: 583 - DNA, 49 bp, Artificial Sequence
  artificial sequence
ctttccagagtttcgtcaccaagagcaacgcccacttgcgggacagagg

SEQ ID NO: 584 - DNA, 39 bp, Artificial Sequence
  artificial sequence
tttgctaaatccagggatagcaagcaaaccaaaatagcg

SEQ ID NO: 585 - DNA, 35 bp, Artificial Sequence
  artificial sequence
tctttgacccccagtaaacagcaaccatcactatc

SEQ ID NO: 586 - DNA, 42 bp, Artificial Sequence
  artificial sequence
gaaccagaccggaaataagtgattattcagcgtttctccctc

SEQ ID NO: 587 - DNA, 41 bp, Artificial Sequence
  artificial sequence
aattgctaaaatcaggtctttgagaatgaccattaaattct

SEQ ID NO: 588 - DNA, 42 bp, Artificial Sequence
  artificial sequence
acaagaggtcattgccgttctaccatcgaaaaacattatgac

SEQ ID NO: 589 - DNA, 35 bp, Artificial Sequence
  artificial sequence
ttaccgaaaacaatgaaatagttaaaatagacacc

SEQ ID NO: 590 - DNA, 42 bp, Artificial Sequence
  artificial sequence
agccctttttaagaaaggaaactccttaagagccataaaggt

SEQ ID NO: 591 - DNA, 42 bp, Artificial Sequence
  artificial sequence
tgccagtttgagccaggcaaagcgcgattttttaagtgcatc

SEQ ID NO: 592 - DNA, 42 bp, Artificial Sequence
  artificial sequence
ggtcagtccagcatcaacggcggattggatcgcacttggtct

SEQ ID NO: 593 - DNA, 42 bp, Artificial Sequence
  artificial sequence
tttagttaataaggcgttaccagagcacgttttcaaatatat

SEQ ID NO: 594 - DNA, 49 bp, Artificial Sequence
  artificial sequence
acctaaatttaaataatgctgatgcaaagctggtacgttatatcgccat

SEQ ID NO: 595 - DNA, 35 bp, Artificial Sequence
  artificial sequence
aaaatcaacccttgcttctgtaaatcgtatagtga

SEQ ID NO: 596 - DNA, 35 bp, Artificial Sequence
  artificial sequence
atgcggcttcgcgtgtaccgaggaagggaggcggt

SEQ ID NO: 597 - DNA, 49 bp, Artificial Sequence
  artificial sequence
gtcataccggggcttcagacgatccagcgtgccgggttatcctcacatt

SEQ ID NO: 598 - DNA, 28 bp, Artificial Sequence
  artificial sequence
ttgacgactgagaagtgttttcgttgta

SEQ ID NO: 599 - DNA, 42 bp, Artificial Sequence
  artificial sequence
cacgaccagtaatagaatacgaaataccattaattaggattt

SEQ ID NO: 600 - DNA, 35 bp, Artificial Sequence
  artificial sequence
ccaaccaggaataagaataaacagaacgaaagtac

SEQ ID NO: 601 - DNA, 35 bp, Artificial Sequence
  artificial sequence
acaacatttaggaaagtgaatatcaagacagatga

SEQ ID NO: 602 - DNA, 42 bp, Artificial Sequence
  artificial sequence
gcctgtaaaggaatttcggtcgctgaccatcggttttgaaaa

SEQ ID NO: 603 - DNA, 45 bp, Artificial Sequence
  artificial sequence
tgtaccgtcgtttaccagacgacgataaccaatagtgtatgggat

SEQ ID NO: 604 - DNA, 42 bp, Artificial Sequence
  artificial sequence
accaccctttgcaaaagaagttttgccaccaccctctcagaa

SEQ ID NO: 605 - DNA, 35 bp, Artificial Sequence
  artificial sequence
gcccgaaactgcggcaggagttgaatttccagagc

SEQ ID NO: 606 - DNA, 40 bp, Artificial Sequence
  artificial sequence
agtcagagctttaaatggtcagcgagctcatacaggcaag

SEQ ID NO: 607 - DNA, 40 bp, Artificial Sequence
  artificial sequence
atgtaccccggtattgtaagacagtcattcaaacaaggat

SEQ ID NO: 608 - DNA, 35 bp, Artificial Sequence
  artificial sequence
acaagaaaaccaataaaatacgcggttttgaagcc

SEQ ID NO: 609 - DNA, 42 bp, Artificial Sequence
  artificial sequence
cgcatcgtaacccaaagtcagcctgtagttaccaacccagct

SEQ ID NO: 610 - DNA, 42 bp, Artificial Sequence
  artificial sequence
tgggataaacccgtgggggatttgtaaagccgccacgggaac

SEQ ID NO: 611 - DNA, 42 bp, Artificial Sequence
  artificial sequence
accagcttacggctgcgcttttaaacgatacatcgaacttaa

SEQ ID NO: 612 - DNA, 28 bp, Artificial Sequence
  artificial sequence
cttaggtgctgagaagagtcacgctatt

SEQ ID NO: 613 - DNA, 28 bp, Artificial Sequence
  artificial sequence
tttttaacctccggcttacacttaatta

SEQ ID NO: 614 - DNA, 37 bp, Artificial Sequence
  artificial sequence
gcactctgtggtggtctgagaaatcgtttaaaacatc

SEQ ID NO: 615 - DNA, 42 bp, Artificial Sequence
  artificial sequence
ccaccgagtaaacataatgcgccgctaccaccacaccctaaa

SEQ ID NO: 616 - DNA, 39 bp, Artificial Sequence
  artificial sequence
gattaaagggactgagtagatggccagggcgagtttgcc

SEQ ID NO: 617 - DNA, 35 bp, Artificial Sequence
  artificial sequence
tcaatcgcagaacagccacgcatatcaaggaaggt

SEQ ID NO: 618 - DNA, 35 bp, Artificial Sequence
  artificial sequence
aaagtacggtaaaatacgtaagactaaagttaaag

SEQ ID NO: 619 - DNA, 42 bp, Artificial Sequence
  artificial sequence
acaacatgtgcctatcgggaaacctgtccggggagttagaac

SEQ ID NO: 620 - DNA, 42 bp, Artificial Sequence
  artificial sequence
acgccaagcattccacagacgttaataaaatgcagacgtaac

SEQ ID NO: 621 - DNA, 35 bp, Artificial Sequence
  artificial sequence
catagtagtacaaataaagttttgtcgtaggaatt

SEQ ID NO: 622 - DNA, 28 bp, Artificial Sequence
  artificial sequence
attaagattcggtccagaaccgccaccc

SEQ ID NO: 623 - DNA, 35 bp, Artificial Sequence
  artificial sequence
agaggcttcattttaggaggtttagtacaggtgta

SEQ ID NO: 624 - DNA, 35 bp, Artificial Sequence
  artificial sequence
aaaatgtaattcgagcttctcagaaccggaggggg

SEQ ID NO: 625 - DNA, 35 bp, Artificial Sequence
  artificial sequence
gtccaatagacttcccaacaggtcaggagttttgc

SEQ ID NO: 626 - DNA, 35 bp, Artificial Sequence
  artificial sequence
ataaataaagattagtacctttaattgctaaagga

SEQ ID NO: 627 - DNA, 42 bp, Artificial Sequence
  artificial sequence
ttcattgtatacatggcttttactcctcaagagcgtagcgcg

SEQ ID NO: 628 - DNA, 35 bp, Artificial Sequence
  artificial sequence
ctcaaatagcaaaggataagaggtcattgttttaa

SEQ ID NO: 629 - DNA, 28 bp, Artificial Sequence
  artificial sequence
agaaaacaccctgaatggcttagagctt

SEQ ID NO: 630 - DNA, 47 bp, Artificial Sequence
  artificial sequence
tgtatatgatatctgagtaccctcatatattttttgtaccatagcag

SEQ ID NO: 631 - DNA, 28 bp, Artificial Sequence
  artificial sequence
tatttaatgataatgaacggtaatcgta

SEQ ID NO: 632 - DNA, 42 bp, Artificial Sequence
  artificial sequence
attttttttgagttgcagatagctaaaaacagggaataaccc

SEQ ID NO: 633 - DNA, 42 bp, Artificial Sequence
  artificial sequence
ccatcaacagagagagcgcattagacggtagcagcaaacagc

SEQ ID NO: 634 - DNA, 42 bp, Artificial Sequence
  artificial sequence
tggccttagggtaaaactgaacaccctggtttaaccaatcca

SEQ ID NO: 635 - DNA, 42 bp, Artificial Sequence
  artificial sequence
gagtaacggtcacgcgacagtatcggcccaccgctgttggga

SEQ ID NO: 636 - DNA, 35 bp, Artificial Sequence
  artificial sequence
tccgtgggaacaagctattaccacagcagttgggc

SEQ ID NO: 637 - DNA, 49 bp, Artificial Sequence
  artificial sequence
attgcagggaggtgcagcaaccgcaagaggacttgcggtccggaaaaat

SEQ ID NO: 638 - DNA, 49 bp, Artificial Sequence
  artificial sequence
aatccgcccacgcacggcagcaccgtcgatcctcacgctggccaataga

SEQ ID NO: 639 - DNA, 42 bp, Artificial Sequence
  artificial sequence
ggttgcggtatgaggcgagaaaacttggtgccatccgggcgc

SEQ ID NO: 640 - DNA, 28 bp, Artificial Sequence
  artificial sequence
aaggtttatatgtaagcgatagcttaga

SEQ ID NO: 641 - DNA, 41 bp, Artificial Sequence
  artificial sequence
tgtccactaaatcgttgagtaatcaaaagaatagcttttca

SEQ ID NO: 642 - DNA, 35 bp, Artificial Sequence
  artificial sequence
aattaactataatcgtactatggttgctagcggtc

SEQ ID NO: 643 - DNA, 56 bp, Artificial Sequence
  artificial sequence
ttctttgcagaatcgcacgtataacgtgcgctaggggcgaacggaattacctgaga

SEQ ID NO: 644 - DNA, 42 bp, Artificial Sequence
  artificial sequence
cacttgcttttagacgttagaatcagagttagaaagcgaaag

SEQ ID NO: 645 - DNA, 49 bp, Artificial Sequence
  artificial sequence
aaaaattcctgtaaacgtcaccaatgaaagctgatcatcaataagcaaa

SEQ ID NO: 646 - DNA, 56 bp, Artificial Sequence
  artificial sequence
tattctaagaacgcccaatagccaagtaccgcactcatattagagcgtctcgcgtc

SEQ ID NO: 647 - DNA, 49 bp, Artificial Sequence
  artificial sequence
attgtgtggtttaactcattctaccacattcaactaacgaactgggaag

SEQ ID NO: 648 - DNA, 35 bp, Artificial Sequence
  artificial sequence
gggtatcaaccattcgccattccttatccaatcgg

SEQ ID NO: 649 - DNA, 22 bp, Artificial Sequence
  artificial sequence
ataccattgcaattaacatctg

SEQ ID NO: 650 - DNA, 35 bp, Artificial Sequence
  artificial sequence
ccaccagacctgaaagcgtaaaaagggattgacgc

SEQ ID NO: 651 - DNA, 35 bp, Artificial Sequence
  artificial sequence
agaagtagaattgaaccctcaatcaataccgcctg

SEQ ID NO: 652 - DNA, 22 bp, Artificial Sequence
  artificial sequence
tctgcagaagataaatccttac

SEQ ID NO: 653 - DNA, 52 bp, Artificial Sequence
  artificial sequence
cagttgaaagttagacttttgcccgaacgttgaacgaacaacagtatattac

SEQ ID NO: 654 - DNA, 24 bp, Artificial Sequence
  artificial sequence
cgccagcctacattcattctggcc

SEQ ID NO: 655 - DNA, 27 bp, Artificial Sequence
  artificial sequence
tttttacttagcacagaccaggcgttt

SEQ ID NO: 656 - DNA, 29 bp, Artificial Sequence
  artificial sequence
attgggctgaattaccttatgcgattttt

SEQ ID NO: 657 - DNA, 33 bp, Artificial Sequence
  artificial sequence
acggtgtcggaacgcgcgacctgctccatgttt

SEQ ID NO: 658 - DNA, 38 bp, Artificial Sequence
  artificial sequence
tttccagaacgagtagtaagccctgacgagaaacattt

SEQ ID NO: 659 - DNA, 29 bp, Artificial Sequence
  artificial sequence
tttcataggctggctgaccttcaaggctt

SEQ ID NO: 660 - DNA, 47 bp, Artificial Sequence
  artificial sequence
tttattcatcagttgagattattacatcattataccagtcatcattg

SEQ ID NO: 661 - DNA, 27 bp, Artificial Sequence
  artificial sequence
tttttaagaactggcggtagaaagttt

SEQ ID NO: 662 - DNA, 47 bp, Artificial Sequence
  artificial sequence
ataaccctaacactgacgttagtaaatgagaatagccgatagttttt

SEQ ID NO: 663 - DNA, 45 bp, Artificial Sequence
  artificial sequence
ccagtaacagttaatgcgtatagcccggaatcgccacccagagcc

SEQ ID NO: 664 - DNA, 29 bp, Artificial Sequence
  artificial sequence
tttgcgccgacacagcgaaagacattgag

SEQ ID NO: 665 - DNA, 35 bp, Artificial Sequence
  artificial sequence
gagtaaccaaataagacgattggccttgatagaag

SEQ ID NO: 666 - DNA, 42 bp, Artificial Sequence
  artificial sequence
cattatacactaaaacactcagaaagaggcaaaagaataccc

SEQ ID NO: 667 - DNA, 38 bp, Artificial Sequence
  artificial sequence
tccccggaaccagagccaccaccgcaggtcaatcctca

SEQ ID NO: 668 - DNA, 31 bp, Artificial Sequence
  artificial sequence
aacttgcatcggaacgagggtagcctaaaac

SEQ ID NO: 669 - DNA, 31 bp, Artificial Sequence
  artificial sequence
tcaggattcacaaaagtgcccgtataacaga

SEQ ID NO: 670 - DNA, 38 bp, Artificial Sequence
  artificial sequence
ccgccacgatataacccctgcatcaaaatcacctacat

SEQ ID NO: 671 - DNA, 45 bp, Artificial Sequence
  artificial sequence
caccgaacagttaatgcgtatagcccggaatcgccacccagagcc

SEQ ID NO: 672 - DNA, 31 bp, Artificial Sequence
  artificial sequence
tcctcgcatcggaacgagggtagcctaaaac

SEQ ID NO: 673 - DNA, 49 bp, Artificial Sequence
  artificial sequence
ataaccctaacactgacgttagtaaatgagaatagccgatagttaattt

SEQ ID NO: 674 - DNA, 38 bp, Artificial Sequence
  artificial sequence
ccgccacgatataacccctgcatcaaaatcacccacca

SEQ ID NO: 675 - DNA, 31 bp, Artificial Sequence
  artificial sequence
ctctggcgccgacacagcgaaagacaattaa

SEQ ID NO: 676 - DNA, 38 bp, Artificial Sequence
  artificial sequence
gccgcggaaccagagccaccaccgcaggtcaatcctca

SEQ ID NO: 677 - DNA, 35 bp, Artificial Sequence
  artificial sequence
gagtaaccaaataagacgattggccttgatgccac

SEQ ID NO: 678 - DNA, 42 bp, Artificial Sequence
  artificial sequence
aggagtacactaaaacactcagaaagaggcaaaagaagttga

SEQ ID NO: 679 - DNA, 31 bp, Artificial Sequence
  artificial sequence
gaaccattcacaaaagtgcccgtatagaacc

SEQ ID NO: 680 - DNA, 42 bp, Artificial Sequence
  artificial sequence
tcttaccgggaggtggtattctaagaaccaagcaaaaccaag

SEQ ID NO: 681 - DNA, 28 bp, Artificial Sequence
  artificial sequence
tattggggttgcagcaagcaaaagggac

SEQ ID NO: 682 - DNA, 28 bp, Artificial Sequence
  artificial sequence
agaggcgggtaaccgttgtagtccagaa

SEQ ID NO: 683 - DNA, 42 bp, Artificial Sequence
  artificial sequence
gcattaaacccttcttacattggcagatcaggaaaccttgct

SEQ ID NO: 684 - DNA, 44 bp, Artificial Sequence
  artificial sequence
ctgtcgtacttgccataatcacgccagaatcctgattatggttg

SEQ ID NO: 685 - DNA, 28 bp, Artificial Sequence
  artificial sequence
ctcactgtattttttaaaaataccgaac

SEQ ID NO: 686 - DNA, 28 bp, Artificial Sequence
  artificial sequence
taatgagaggatgccgggttatggtgct

SEQ ID NO: 687 - DNA, 49 bp, Artificial Sequence
  artificial sequence
gggtgccatggtcagggtaccgagctcgctcagaatgcggcgggccgtt

SEQ ID NO: 688 - DNA, 35 bp, Artificial Sequence
  artificial sequence
aagcatagtgaaattcctcacagttgagttcacgg

SEQ ID NO: 689 - DNA, 34 bp, Artificial Sequence
  artificial sequence
acatacgcatcagtaaacattgggtaaaggtttc

SEQ ID NO: 690 - DNA, 28 bp, Artificial Sequence
  artificial sequence
cagggttggcttagtcccttagaatcct

SEQ ID NO: 691 - DNA, 49 bp, Artificial Sequence
  artificial sequence
cttcgctaaccaggttccggcaccgcttggcgcatgggatagtgcagaa

SEQ ID NO: 692 - DNA, 49 bp, Artificial Sequence
  artificial sequence
aagggcgccattcaaagatcgcactccatgccagtaaacggcaacaata

SEQ ID NO: 693 - DNA, 35 bp, Artificial Sequence
  artificial sequence
agcattaacatcacggagacaggcattttttaacc

SEQ ID NO: 694 - DNA, 42 bp, Artificial Sequence
  artificial sequence
atcaattaattagcacattatgaccctgcgcaagggtaggta

SEQ ID NO: 695 - DNA, 42 bp, Artificial Sequence
  artificial sequence
tttagctctgaacagaagcgcattagacatccaaaataaaca

SEQ ID NO: 696 - DNA, 42 bp, Artificial Sequence
  artificial sequence
tcgcaaaagagggtagagaataacataattgtttagcctaat

SEQ ID NO: 697 - DNA, 42 bp, Artificial Sequence
  artificial sequence
agtttgaatcagaggaagcccttcagcctttacagaattgag

SEQ ID NO: 698 - DNA, 28 bp, Artificial Sequence
  artificial sequence
acggtgtaatataattgataagaggtca

SEQ ID NO: 699 - DNA, 47 bp, Artificial Sequence
  artificial sequence
tgcaaattaagaataaatcaacagttcagaaaatagtaaaaaacgtc

SEQ ID NO: 700 - DNA, 28 bp, Artificial Sequence
  artificial sequence
tcatcaacccaaatgcttgagatggttt

SEQ ID NO: 701 - DNA, 35 bp, Artificial Sequence
  artificial sequence
ggcgcattgctcatccagaacgagtagtatgcgat

SEQ ID NO: 702 - DNA, 49 bp, Artificial Sequence
  artificial sequence
cggtgtattgttgaggcaggtttaccgttccagttagtttgcaccagag

SEQ ID NO: 703 - DNA, 35 bp, Artificial Sequence
  artificial sequence
tgaccaatattctgtgcccgtataaacattgatga

SEQ ID NO: 704 - DNA, 49 bp, Artificial Sequence
  artificial sequence
tcaatcataagaggggtcagtgccttgaggtaatacattaaattttcgg

SEQ ID NO: 705 - DNA, 28 bp, Artificial Sequence
  artificial sequence
gccggaagagaagggggttgatataagt

SEQ ID NO: 706 - DNA, 49 bp, Artificial Sequence
  artificial sequence
aaatccgcgacctgggttttgctcagtaaaacacttgtgtcggcgggat

SEQ ID NO: 707 - DNA, 42 bp, Artificial Sequence
  artificial sequence
ccaacagagatagatgaatcgtctttgataaaagaggatttt

SEQ ID NO: 708 - DNA, 40 bp, Artificial Sequence
  artificial sequence
tattagtttaattgctggtcaaaggttaataatacatttg

SEQ ID NO: 709 - DNA, 35 bp, Artificial Sequence
  artificial sequence
cgctcacaattctatgttcttcgcgtcctctgcca

SEQ ID NO: 710 - DNA, 41 bp, Artificial Sequence
  artificial sequence
gtgaatttcagagtttgagcaaaagaaaaacagtacatatg

SEQ ID NO: 711 - DNA, 28 bp, Artificial Sequence
  artificial sequence
aatcataggtctgaaacgacgaaacaaa

SEQ ID NO: 712 - DNA, 28 bp, Artificial Sequence
  artificial sequence
gagactaatagcgatagcttaataacct

SEQ ID NO: 713 - DNA, 42 bp, Artificial Sequence
  artificial sequence
caaagcgccattcgatcggtgagtaacaacgccatcgcatta

SEQ ID NO: 714 - DNA, 42 bp, Artificial Sequence
  artificial sequence
ggcaaagctactaaaatatgaagagatctggagcaaacaaga

SEQ ID NO: 715 - DNA, 49 bp, Artificial Sequence
  artificial sequence
aagcctcagagcgagaattaaatattttcagctactcaagattcagata

SEQ ID NO: 716 - DNA, 35 bp, Artificial Sequence
  artificial sequence
cgctaatccattagacgcagttaagcgaacctccc

SEQ ID NO: 717 - DNA, 40 bp, Artificial Sequence
  artificial sequence
gcttaattgctgctggaagaaagcggtaccctggaatccc

SEQ ID NO: 718 - DNA, 40 bp, Artificial Sequence
  artificial sequence
acaaagcaggctggttgagatataacgcccagacgacgat

SEQ ID NO: 719 - DNA, 40 bp, Artificial Sequence
  artificial sequence
ttcggaacctatctttgaattggcctagagccgagccgcc

SEQ ID NO: 720 - DNA, 35 bp, Artificial Sequence
  artificial sequence
agcgattttgtatcgcgaaaggatatatgatagtt

SEQ ID NO: 721 - DNA, 26 bp, Artificial Sequence
  artificial sequence
gctggtttgcccataaatcttccagt

SEQ ID NO: 722 - DNA, 35 bp, Artificial Sequence
  artificial sequence
accagtaagttaccgccagccattgcaatcaccag

SEQ ID NO: 723 - DNA, 35 bp, Artificial Sequence
  artificial sequence
caatcgtctgaaattacctactagaagaagggcgc

SEQ ID NO: 724 - DNA, 28 bp, Artificial Sequence
  artificial sequence
gaaccctcgtggcacagacaacccgctt

SEQ ID NO: 725 - DNA, 28 bp, Artificial Sequence
  artificial sequence
gatcccctagctgtttcctgtaagtgta

SEQ ID NO: 726 - DNA, 49 bp, Artificial Sequence
  artificial sequence
gacgcagaaacacccagcgccatgtttaaacaatcagttaaatcctcat

SEQ ID NO: 727 - DNA, 40 bp, Artificial Sequence
  artificial sequence
gaagggatagcttttgccgaaaaaattttggatcggtggt

SEQ ID NO: 728 - DNA, 35 bp, Artificial Sequence
  artificial sequence
gaagagtgtaatcaatatatgtgagtgagattaag

SEQ ID NO: 729 - DNA, 48 bp, Artificial Sequence
  artificial sequence
attttagttaatttgttgggttatataaaagttggaaaagcccaacag

SEQ ID NO: 730 - DNA, 42 bp, Artificial Sequence
  artificial sequence
cgagaaatttgaaataccggtgtagatgctagacaaagaacg

SEQ ID NO: 731 - DNA, 42 bp, Artificial Sequence
  artificial sequence
ctcaggggctgcgcacaataaatcatatttgcgggaatcggc

SEQ ID NO: 732 - DNA, 42 bp, Artificial Sequence
  artificial sequence
taaatcggttgtaaccctcatatatttatcccaggataaagc

SEQ ID NO: 733 - DNA, 42 bp, Artificial Sequence
  artificial sequence
aatagcaatagctaagatagccaaaagaccgacttaaatatt

SEQ ID NO: 734 - DNA, 35 bp, Artificial Sequence
  artificial sequence
acaatgattaagcccaataatacagttgggcaaca

SEQ ID NO: 735 - DNA, 42 bp, Artificial Sequence
  artificial sequence
tttaattcaacagggcccgaaaggccggatgtttagactgga

SEQ ID NO: 736 - DNA, 41 bp, Artificial Sequence
  artificial sequence
aatttgaccggatattcattagagtaatacaggtaaggcat

SEQ ID NO: 737 - DNA, 41 bp, Artificial Sequence
  artificial sequence
atagcggctgagactcctcaacgaggcgtaggaacgcattc

SEQ ID NO: 738 - DNA, 49 bp, Artificial Sequence
  artificial sequence
ggcggataagtgccggaggttgaaccgcgaacaacaatgaattttctgt

SEQ ID NO: 739 - DNA, 23 bp, Artificial Sequence
  artificial sequence
aggcaaaagaatactcgactttt

SEQ ID NO: 740 - DNA, 42 bp, Artificial Sequence
  artificial sequence
ggcaccaacctaaattccattcggctacaaatctcgtatcgg

SEQ ID NO: 741 - DNA, 42 bp, Artificial Sequence
  artificial sequence
gaagaaatctaattattaatcgtattaaatcctgaaactaat

SEQ ID NO: 742 - DNA, 35 bp, Artificial Sequence
  artificial sequence
acaccgcaaaactgatagccctaaaacaggcggtc

SEQ ID NO: 743 - DNA, 33 bp, Artificial Sequence
  artificial sequence
gcggatcaaactcgcacagtcatcaaccagctt

SEQ ID NO: 744 - DNA, 42 bp, Artificial Sequence
  artificial sequence
ctgctcactcacggcggaatttgtgagaggaacgggttccgg

SEQ ID NO: 745 - DNA, 23 bp, Artificial Sequence
  artificial sequence
ccagcagttgggcgcaccgtggt

SEQ ID NO: 746 - DNA, 42 bp, Artificial Sequence
  artificial sequence
gtaaatctgaaaaccctttttaacctccttcccagaattaat

SEQ ID NO: 747 - DNA, 26 bp, Artificial Sequence
  artificial sequence
gtcgctatttaacaaaaacagaaata

SEQ ID NO: 748 - DNA, 42 bp, Artificial Sequence
  artificial sequence
tctgaaagaataaattctgataaagtaccgacattttaattg

SEQ ID NO: 749 - DNA, 42 bp, Artificial Sequence
  artificial sequence
ttaatggacttttttaaatgctgatgcagggatgttgcgtta

SEQ ID NO: 750 - DNA, 35 bp, Artificial Sequence
  artificial sequence
gacgacgacagtgatgagaaaaagaaaacagaaaa

SEQ ID NO: 751 - DNA, 42 bp, Artificial Sequence
  artificial sequence
tttttagaccaaaaaaaattaagcaatagctgaaaagctgat

SEQ ID NO: 752 - DNA, 35 bp, Artificial Sequence
  artificial sequence
cgattttaaacaggccctgaacaaagtctggtcaa

SEQ ID NO: 753 - DNA, 42 bp, Artificial Sequence
  artificial sequence
agtaagctcttaccagataacccacaaggaacgagagaaaat

SEQ ID NO: 754 - DNA, 42 bp, Artificial Sequence
  artificial sequence
ttcaaagcgtttttgcggatggagcaagaaagaaggaaaccg

SEQ ID NO: 755 - DNA, 49 bp, Artificial Sequence
  artificial sequence
aaccagagcgttttgtagcaccaatactgcggaatcgtcacacagcaaa

SEQ ID NO: 756 - DNA, 42 bp, Artificial Sequence
  artificial sequence
caaactcgctcctttgctgtagctcaacatgttaagagtacc

SEQ ID NO: 757 - DNA, 47 bp, Artificial Sequence
  artificial sequence
aatcataataaaaaaccatgccagagggggtaacgagcaacactatc

SEQ ID NO: 758 - DNA, 28 bp, Artificial Sequence
  artificial sequence
actggctagaaacatcagtgaataaggc

SEQ ID NO: 759 - DNA, 42 bp, Artificial Sequence
  artificial sequence
catacatggcttgttaatgcccccgccctgacgcataagcgt

SEQ ID NO: 760 - DNA, 42 bp, Artificial Sequence
  artificial sequence
gtgtactgtaacagaaacatgaaagtattaagggaaaataaa

SEQ ID NO: 761 - DNA, 43 bp, Artificial Sequence
  artificial sequence
taggtgccaccctcagcggatttgctaaacaactcccagccct

SEQ ID NO: 762 - DNA, 42 bp, Artificial Sequence
  artificial sequence
gtactcagtcgagaattaggattagcggctccatgactgagt

SEQ ID NO: 763 - DNA, 26 bp, Artificial Sequence
  artificial sequence
tcatgaggaagtacgaaaggaccccc

SEQ ID NO: 764 - DNA, 29 bp, Artificial Sequence
  artificial sequence
caataattgcgcgtagagcgggatttaga

SEQ ID NO: 765 - DNA, 23 bp, Artificial Sequence
  artificial sequence
ccttgagattttgacgaccagca

SEQ ID NO: 766 - DNA, 42 bp, Artificial Sequence
  artificial sequence
gagagccgtaacatctttacaaacaatttcaatagtctaaaa

SEQ ID NO: 767 - DNA, 42 bp, Artificial Sequence
  artificial sequence
gcggcgcacaaagacgccgggcgagaagtattagatatcatt

SEQ ID NO: 768 - DNA, 42 bp, Artificial Sequence
  artificial sequence
gcctgtggcggaatcaggcgctttcgcacgggtcacaaatcg

SEQ ID NO: 769 - DNA, 42 bp, Artificial Sequence
  artificial sequence
tccagcgtgattatccagcatcagcgggctggtaacccttac

SEQ ID NO: 770 - DNA, 42 bp, Artificial Sequence
  artificial sequence
accttttatatcaaaacgtcagatgaatatacaaaggttaga

SEQ ID NO: 771 - DNA, 46 bp, Artificial Sequence
  artificial sequence
tcctctaggtgaattatcaccgtcaactggcacaaacgttagattt

SEQ ID NO: 772 - DNA, 42 bp, Artificial Sequence
  artificial sequence
gttgggataatcagggcttttgcaaaagtcgtttacaaaagg

SEQ ID NO: 773 - DNA, 37 bp, Artificial Sequence
  artificial sequence
tctgaatcagacgaagaggacagatgaatttgcctat

SEQ ID NO: 774 - DNA, 42 bp, Artificial Sequence
  artificial sequence
cgcagtctgtagcgttcataatcaaaatccctcagccgccag

SEQ ID NO: 775 - DNA, 35 bp, Artificial Sequence
  artificial sequence
ctaaaagataataattcgaggtgcagacgttagta

SEQ ID NO: 776 - DNA, 26 bp, Artificial Sequence
  artificial sequence
tcaaatccagtcgggaaacaagaata

SEQ ID NO: 777 - DNA, 37 bp, Artificial Sequence
  artificial sequence
tatcaaaaggagcactaacagtgttttttgctgaacc

SEQ ID NO: 778 - DNA, 35 bp, Artificial Sequence
  artificial sequence
ccagcggtgttcagctgttgccctgcgggtcattg

SEQ ID NO: 779 - DNA, 35 bp, Artificial Sequence
  artificial sequence
tacaagctgaccgtgtgataaataaacatcgagcc

SEQ ID NO: 780 - DNA, 49 bp, Artificial Sequence
  artificial sequence
cagctttcagctggcgaaaggaatccaatcgcaggtgccggaattacgc

SEQ ID NO: 781 - DNA, 28 bp, Artificial Sequence
  artificial sequence
catcaacgtctggccgttaatattttgt

SEQ ID NO: 782 - DNA, 35 bp, Artificial Sequence
  artificial sequence
aaatttttattttaaatgcaaccaatcacgtaaaa

SEQ ID NO: 783 - DNA, 42 bp, Artificial Sequence
  artificial sequence
acggctgttaacgtgccggacttgtagacacgcaatataatc

SEQ ID NO: 784 - DNA, 28 bp, Artificial Sequence
  artificial sequence
tataagtgcaggaaacgcaatttagagc

SEQ ID NO: 785 - DNA, 35 bp, Artificial Sequence
  artificial sequence
ttcgtgcaccctcatagtaccgccacccactacca

SEQ ID NO: 786 - DNA, 44 bp, Artificial Sequence
  artificial sequence
actacgtaaaccgtagtgttgaaaagaatagcccgatggtccac

SEQ ID NO: 787 - DNA, 42 bp, Artificial Sequence
  artificial sequence
catcacgcaaatcgtaaacaggaggccgtagaatcaaccacc

SEQ ID NO: 788 - DNA, 56 bp, Artificial Sequence
  artificial sequence
caccgagttagtaactatcggaacgctcatggaaaggattattgacctgaaagcgt

SEQ ID NO: 789 - DNA, 49 bp, Artificial Sequence
  artificial sequence
tatctttccctcaaaatgaaataaaacagaggtgatcgccatgaatggc

SEQ ID NO: 790 - DNA, 35 bp, Artificial Sequence
  artificial sequence
ttaacggcatcattgttgcggtatgagcctcaatc

SEQ ID NO: 791 - DNA, 49 bp, Artificial Sequence
  artificial sequence
actggtgtgccggtactgcgctcataccgggggttgtgagcctgttatc

SEQ ID NO: 792 - DNA, 43 bp, Artificial Sequence
  artificial sequence
aacggtgctcgtcaacgatgaagggtaaggcgaaacgcacaca

SEQ ID NO: 793 - DNA, 35 bp, Artificial Sequence
  artificial sequence
gcagcctcgtggtgctggtctgcaccgttatactt

SEQ ID NO: 794 - DNA, 28 bp, Artificial Sequence
  artificial sequence
tcgtctcgtcgctgcaaacgccgacata

SEQ ID NO: 795 - DNA, 35 bp, Artificial Sequence
  artificial sequence
gaggcgatttacatcgggagacaggtttaattatt

SEQ ID NO: 796 - DNA, 35 bp, Artificial Sequence
  artificial sequence
accaagtacggattcgcctgaaaaagaaattgcgt

SEQ ID NO: 797 - DNA, 36 bp, Artificial Sequence
  artificial sequence
tagggcgctttgaattaataattactagagtaacgc

SEQ ID NO: 798 - DNA, 42 bp, Artificial Sequence
  artificial sequence
aattcgcattaaatccgtaatcgtaaccgtgcatcgccagct

SEQ ID NO: 799 - DNA, 28 bp, Artificial Sequence
  artificial sequence
aataggaacccgtcggattcctgttggg

SEQ ID NO: 800 - DNA, 49 bp, Artificial Sequence
  artificial sequence
gctatcagtcaaataaaagggagcctttatttcaataatactcaggcaa

SEQ ID NO: 801 - DNA, 35 bp, Artificial Sequence
  artificial sequence
tttgaagccttaaaaattttattacaaataagaaa

SEQ ID NO: 802 - DNA, 28 bp, Artificial Sequence
  artificial sequence
gacttgcaacgctaacgagttatacatt

SEQ ID NO: 803 - DNA, 35 bp, Artificial Sequence
  artificial sequence
agtttattaccagcgccaaagggaaggtgagccat

SEQ ID NO: 804 - DNA, 35 bp, Artificial Sequence
  artificial sequence
cggaataacatacagaatacccgaacaaagttacc

SEQ ID NO: 805 - DNA, 42 bp, Artificial Sequence
  artificial sequence
cgcaaaggcgacatttaaatattcattactattataaagaaa

SEQ ID NO: 806 - DNA, 45 bp, Artificial Sequence
  artificial sequence
agtaagagaatgaccggaacaacattattcttgacaagttaaata

SEQ ID NO: 807 - DNA, 49 bp, Artificial Sequence
  artificial sequence
aattacggaaagattctacgtttgtgaattaccttaaattggcaacgta

SEQ ID NO: 808 - DNA, 21 bp, Artificial Sequence
  artificial sequence
cattgacaggagcacaccgga

SEQ ID NO: 809 - DNA, 28 bp, Artificial Sequence
  artificial sequence
caccacctgatatttggaaagtacagga

SEQ ID NO: 810 - DNA, 28 bp, Artificial Sequence
  artificial sequence
gccgccacaccctcagagccattgcccc

SEQ ID NO: 811 - DNA, 36 bp, Artificial Sequence
  artificial sequence
cacagaaccctcagatctagcaagcccaacagacgg

SEQ ID NO: 812 - DNA, 42 bp, Artificial Sequence
  artificial sequence
tacaaataaagttttgtcgtctttcaagagttaaagcaccag

SEQ ID NO: 813 - DNA, 35 bp, Artificial Sequence
  artificial sequence
ttgcaggtttcttaaacagctgcttgctttttttc

SEQ ID NO: 814 - DNA, 49 bp, Artificial Sequence
  artificial sequence
agacaggcgtataataatgcgccgctacactcaaataacatcgccagct

SEQ ID NO: 815 - DNA, 26 bp, Artificial Sequence
  artificial sequence
agattagagccgcgacaacttttaaa

SEQ ID NO: 816 - DNA, 44 bp, Artificial Sequence
  artificial sequence
aggatttcggaaaggaattgagggttggcaccacgctagtatta

SEQ ID NO: 817 - DNA, 42 bp, Artificial Sequence
  artificial sequence
gtacctattattcatttcaattaccttagcaaccgcgtaaca

SEQ ID NO: 818 - DNA, 26 bp, Artificial Sequence
  artificial sequence
agaatcgccataagagaattccagac

SEQ ID NO: 819 - DNA, 42 bp, Artificial Sequence
  artificial sequence
aatttagaacttcctgtaattcttaccagtacgccaacatgt

SEQ ID NO: 820 - DNA, 49 bp, Artificial Sequence
  artificial sequence
aatttttaaacagggataagtcctgaacggctccgtgggaacttgaggg

SEQ ID NO: 821 - DNA, 42 bp, Artificial Sequence
  artificial sequence
agcaaatagttgctaaatgccggagagtgaacggtaatagca

SEQ ID NO: 822 - DNA, 49 bp, Artificial Sequence
  artificial sequence
tagaaggcatcgtatcattccaagaacgttgccagtcctgaataacctg

SEQ ID NO: 823 - DNA, 49 bp, Artificial Sequence
  artificial sequence
cctcaaatagcgtccattaccattagcaagacttccaaaaagctaaagt

SEQ ID NO: 824 - DNA, 42 bp, Artificial Sequence
  artificial sequence
tgctttaaaaaatcaggtcttattgcataaatatcccggaag

SEQ ID NO: 825 - DNA, 49 bp, Artificial Sequence
  artificial sequence
ataacccaagttttcgatagcagcaccgagaaaaatcatcagctgacct

SEQ ID NO: 826 - DNA, 44 bp, Artificial Sequence
  artificial sequence
aaaaaccacactaatgcagatacttaggaatcaggactttaaga

SEQ ID NO: 827 - DNA, 28 bp, Artificial Sequence
  artificial sequence
accgcctcaccggactttagcgtcagac

SEQ ID NO: 828 - DNA, 49 bp, Artificial Sequence
  artificial sequence
accctcaccatcttcgttttcatcggcagccagaacacaaacaccgaac

SEQ ID NO: 829 - DNA, 19 bp, Artificial Sequence
  artificial sequence
catagttagcgtatgggat

SEQ ID NO: 830 - DNA, 42 bp, Artificial Sequence
  artificial sequence
aacgatcctacaacgcctgtaccatgtaagagccatatcacc

SEQ ID NO: 831 - DNA, 41 bp, Artificial Sequence
  artificial sequence
gcttgatgtagcggtcacgcagggttgctatcaggtttgcg

SEQ ID NO: 832 - DNA, 26 bp, Artificial Sequence
  artificial sequence
ctttgacgagcaaacggtagtgaggc

SEQ ID NO: 833 - DNA, 44 bp, Artificial Sequence
  artificial sequence
gaggtgtcagatgatggcaatgcggcctttagtgagcacgcgtg

SEQ ID NO: 834 - DNA, 28 bp, Artificial Sequence
  artificial sequence
atggaaggaatgccaacggcaggtcagc

SEQ ID NO: 835 - DNA, 49 bp, Artificial Sequence
  artificial sequence
gccatccacgtcagccggccagagcacacgatgctaaaaagctaaattt

SEQ ID NO: 836 - DNA, 49 bp, Artificial Sequence
  artificial sequence
agattttaacaatatacaaaatcgcgcacatcaagttgaatttgcttct

SEQ ID NO: 837 - DNA, 49 bp, Artificial Sequence
  artificial sequence
agtaatatttaacaataaagccaacgcttgtttaggttaaatcctaaat

SEQ ID NO: 838 - DNA, 42 bp, Artificial Sequence
  artificial sequence
taaattgtagcagaggcatttacatgttcagctaagtcacgt

SEQ ID NO: 839 - DNA, 42 bp, Artificial Sequence
  artificial sequence
aaatattcgcgcctgtttatcggattgagtgagcgcgggcct

SEQ ID NO: 840 - DNA, 28 bp, Artificial Sequence
  artificial sequence
aagattgtataagctaaaattcaaaaat

SEQ ID NO: 841 - DNA, 35 bp, Artificial Sequence
  artificial sequence
gccccaagttaaatcagcttcattgccttgataat

SEQ ID NO: 842 - DNA, 42 bp, Artificial Sequence
  artificial sequence
gtcaatccgagcatgtagaaatgcctgaccgttctaggtggc

SEQ ID NO: 843 - DNA, 49 bp, Artificial Sequence
  artificial sequence
ctagcatgaatcgaggtagctatttttgtattcaagtaatgtataaaaa

SEQ ID NO: 844 - DNA, 42 bp, Artificial Sequence
  artificial sequence
cattaacatcgagaagcgaggcgttttgaaaattcaattatt

SEQ ID NO: 845 - DNA, 49 bp, Artificial Sequence
  artificial sequence
gacggaatatggtttttgtcacaatcaaatgttagtgattaataagaaa

SEQ ID NO: 846 - DNA, 28 bp, Artificial Sequence
  artificial sequence
accgattgagggagacaaaaggacacca

SEQ ID NO: 847 - DNA, 49 bp, Artificial Sequence
  artificial sequence
ccaaaatagcgagatagcgacagaatcaataccagtaccacacagacca

SEQ ID NO: 848 - DNA, 28 bp, Artificial Sequence
  artificial sequence
cttattagcgtttggaaccgcccagaac

SEQ ID NO: 849 - DNA, 42 bp, Artificial Sequence
  artificial sequence
tttatcatgatacctcggtcgctgaggccgtcaccttgagga

SEQ ID NO: 850 - DNA, 35 bp, Artificial Sequence
  artificial sequence
tggcaagcggggaaagccggcatcggaacacccaa

SEQ ID NO: 851 - DNA, 49 bp, Artificial Sequence
  artificial sequence
acacccgggtaatacaatactgccaacgcgcggggattctggtcacacg

SEQ ID NO: 852 - DNA, 35 bp, Artificial Sequence
  artificial sequence
ccgcgctcgtgctttcctcgtattaaaggtctgtc

SEQ ID NO: 853 - DNA, 21 bp, Artificial Sequence
  artificial sequence
gtactgcccgaacgagcatca

SEQ ID NO: 854 - DNA, 28 bp, Artificial Sequence
  artificial sequence
agtttgaagcagcatcaatatcgttgcg

SEQ ID NO: 855 - DNA, 56 bp, Artificial Sequence
  artificial sequence
ttgcggaaacagtgaatcaactgagctaactcacactttaatgcgcgttcgtaatc

SEQ ID NO: 856 - DNA, 35 bp, Artificial Sequence
  artificial sequence
aaccaccagaaggacactctgcctgcagaagcctg

SEQ ID NO: 857 - DNA, 35 bp, Artificial Sequence
  artificial sequence
tatcatcatattcccagtgtcgccccctgagccgg

SEQ ID NO: 858 - DNA, 49 bp, Artificial Sequence
  artificial sequence
ctgattgcccgtaagattgccataacctcaccggaccagtccaaaaaga

SEQ ID NO: 859 - DNA, 50 bp, Artificial Sequence
  artificial sequence
ctgaatatgtacatggtccgtgtggagccgccacggatagactttctata

SEQ ID NO: 860 - DNA, 37 bp, Artificial Sequence
  artificial sequence
accaatgacgaactaacggaatcaggattacaacttt

SEQ ID NO: 861 - DNA, 49 bp, Artificial Sequence
  artificial sequence
acctaccttaatgggatgatggccagtgccaagctttatcaaacgctga

SEQ ID NO: 862 - DNA, 35 bp, Artificial Sequence
  artificial sequence
tgcacgtatttcataaaacaatcacgacgttgtaa

SEQ ID NO: 863 - DNA, 39 bp, Artificial Sequence
  artificial sequence
aggtaaagtaacaccggaatccattaattaatttcatct

SEQ ID NO: 864 - DNA, 49 bp, Artificial Sequence
  artificial sequence
gacgacaataaggctatcatagctgcaaggcgattctatatgcaaatat

SEQ ID NO: 865 - DNA, 35 bp, Artificial Sequence
  artificial sequence
ataatatcccatccaagattccaccatctagtagt

SEQ ID NO: 866 - DNA, 35 bp, Artificial Sequence
  artificial sequence
taatttaatatgtaccccggtgagagtctacaaag

SEQ ID NO: 867 - DNA, 35 bp, Artificial Sequence
  artificial sequence
gctgtctgccatatttgcacccatttggggcgcga

SEQ ID NO: 868 - DNA, 35 bp, Artificial Sequence
  artificial sequence
ttccttaggaatcattaccgcgcccaatataatcg

SEQ ID NO: 869 - DNA, 28 bp, Artificial Sequence
  artificial sequence
ggtattagccgtttttattttcttatcc

SEQ ID NO: 870 - DNA, 45 bp, Artificial Sequence
  artificial sequence
taccgcatacgtctttccagaacgtcaaaaatgaaaatagttgac

SEQ ID NO: 871 - DNA, 42 bp, Artificial Sequence
  artificial sequence
ttgggaaaataacgtaaaggtattcccaattctgcaattgag

SEQ ID NO: 872 - DNA, 44 bp, Artificial Sequence
  artificial sequence
atcaccaaattcgacagaagctttcattccatataaagcttaga

SEQ ID NO: 873 - DNA, 35 bp, Artificial Sequence
  artificial sequence
gtgagaatagaaagcaccctcccgtaacttactta

SEQ ID NO: 874 - DNA, 43 bp, Artificial Sequence
  artificial sequence
tcatacaacagtttcattttcagggactagttttaacccggaa

SEQ ID NO: 875 - DNA, 42 bp, Artificial Sequence
  artificial sequence
acgttgaagaggctctcagcaatcgcctgataaatcatcttt

SEQ ID NO: 876 - DNA, 28 bp, Artificial Sequence
  artificial sequence
taaaggaattgcgaaaccgcccgctttt

SEQ ID NO: 877 - DNA, 42 bp, Artificial Sequence
  artificial sequence
gggcgaagaaccatccctaaagggagcccccgagcatggccc

SEQ ID NO: 878 - DNA, 28 bp, Artificial Sequence
  artificial sequence
cagcaggctggccctgagagacgccagg

SEQ ID NO: 879 - DNA, 35 bp, Artificial Sequence
  artificial sequence
atcaagtactccaaaagagtccggcaaaatccctt

SEQ ID NO: 880 - DNA, 35 bp, Artificial Sequence
  artificial sequence
gggcgctagggcgcttggaaccgtcaaagtggttt

SEQ ID NO: 881 - DNA, 29 bp, Artificial Sequence
  artificial sequence
tttaggtgccgtaaagcactaagaacgtg

SEQ ID NO: 882 - DNA, 38 bp, Artificial Sequence
  artificial sequence
tttagaaagcgaaaggagcgcgagaaaggaagggattt

SEQ ID NO: 883 - DNA, 38 bp, Artificial Sequence
  artificial sequence
tttaacagctgattgccctcaccagtgagacgggcttt

SEQ ID NO: 884 - DNA, 27 bp, Artificial Sequence
  artificial sequence
ttttggttccgaaatcactattaattt

SEQ ID NO: 885 - DNA, 27 bp, Artificial Sequence
  artificial sequence
tttagaacgtggtttttggggtcgttt

SEQ ID NO: 886 - DNA, 36 bp, Artificial Sequence
  artificial sequence
ttctttttcaccgccgaaaatcctgtttgatggttt

SEQ ID NO: 887 - DNA, 32 bp, Artificial Sequence
  artificial sequence
acaggaaaaaaagtacaacggagatataccaa

SEQ ID NO: 888 - DNA, 51 bp, Artificial Sequence
  artificial sequence
gtcagttgccatcgcccacgcataaccacagcatcggaagaggcggtcagt

SEQ ID NO: 889 - DNA, 42 bp, Artificial Sequence
  artificial sequence
aacagagattgccactacgaagcgcgaaacacgctcatggaa

SEQ ID NO: 890 - DNA, 51 bp, Artificial Sequence
  artificial sequence
taaaacagaggtcgagggtagcaaaaacgggtaaaatacgtaaagaaccct

SEQ ID NO: 891 - DNA, 39 bp, Artificial Sequence
  artificial sequence
gcgccgatttaattcaaaaaaaaggctccaaactcgtat

SEQ ID NO: 892 - DNA, 42 bp, Artificial Sequence
  artificial sequence
aaacaattcgacaaaggagcccaatgacaacaagcaaatcaa

SEQ ID NO: 893 - DNA, 35 bp, Artificial Sequence
  artificial sequence
caaaagaatcatcgtccatgtggtgctgcgctggc

SEQ ID NO: 894 - DNA, 28 bp, Artificial Sequence
  artificial sequence
tcatatattagcaataaatcatagatac

SEQ ID NO: 895 - DNA, 42 bp, Artificial Sequence
  artificial sequence
cgttctacggataaaaccaaaatagcgctgcgggataccccg

SEQ ID NO: 896 - DNA, 35 bp, Artificial Sequence
  artificial sequence
aacgcaaaactagcatgtcaatatcaggattcaac

SEQ ID NO: 897 - DNA, 42 bp, Artificial Sequence
  artificial sequence
aattaagcaataaaaattttttaaccctaaacgtacagcgga

SEQ ID NO: 898 - DNA, 35 bp, Artificial Sequence
  artificial sequence
agtagtacaataacacagttgatgctgttcatttt

SEQ ID NO: 899 - DNA, 49 bp, Artificial Sequence
  artificial sequence
aacggtatctggagtcaaatcaccatcaatcggcgcgtttacccagagg

SEQ ID NO: 900 - DNA, 35 bp, Artificial Sequence
  artificial sequence
gaagccttcggttgggtggcatttcattctggaag

SEQ ID NO: 901 - DNA, 49 bp, Artificial Sequence
  artificial sequence
aattgctgaatataattcccattcattgctattacataaacacggggtc

SEQ ID NO: 902 - DNA, 49 bp, Artificial Sequence
  artificial sequence
taaatatttaaattgtgagcgaaactccaacaggtgttttaagatgggc

SEQ ID NO: 903 - DNA, 21 bp, Artificial Sequence
  artificial sequence
ctcgtatgcaagactgtaatt

SEQ ID NO: 904 - DNA, 42 bp, Artificial Sequence
  artificial sequence
ggccttcctgtagcttaaccatcggccttaccctgaggcttg

SEQ ID NO: 905 - DNA, 42 bp, Artificial Sequence
  artificial sequence
cagctttagagagtacctttaccgaaagcatctgctggtgct

SEQ ID NO: 906 - DNA, 42 bp, Artificial Sequence
  artificial sequence
cactgccaataggatagcattcctgtgtgaaattgtaccgag

SEQ ID NO: 907 - DNA, 42 bp, Artificial Sequence
  artificial sequence
atatcgccaggattcatcaacattaaattttgttatccagcc

SEQ ID NO: 908 - DNA, 31 bp, Artificial Sequence
  artificial sequence
aagtttggtattagccaagttgcagaggcga

SEQ ID NO: 909 - DNA, 42 bp, Artificial Sequence
  artificial sequence
cctcagagtgaattacaatgacaacaacagtttccttaatgc

SEQ ID NO: 910 - DNA, 35 bp, Artificial Sequence
  artificial sequence
atcgcacaatcagcagctcaacatgttttttcatt

SEQ ID NO: 911 - DNA, 35 bp, Artificial Sequence
  artificial sequence
aaccgccgtttatccacgcataaccgatctaaaga

SEQ ID NO: 912 - DNA, 42 bp, Artificial Sequence
  artificial sequence
actattaataaataattctgcatttcgcaaatggtgcattaa

SEQ ID NO: 913 - DNA, 49 bp, Artificial Sequence
  artificial sequence
aaaaatcctcaaatccatatactgtttagctatattcaattctaacgcc

SEQ ID NO: 914 - DNA, 35 bp, Artificial Sequence
  artificial sequence
ataaatcccgctttgcatcggactcctccgcctgg

SEQ ID NO: 915 - DNA, 35 bp, Artificial Sequence
  artificial sequence
aaacgagaatgaccagctttctggtgtattcgagc

SEQ ID NO: 916 - DNA, 42 bp, Artificial Sequence
  artificial sequence
accctcagatataagtatagcctatttcctttttcgtaatgg

SEQ ID NO: 917 - DNA, 35 bp, Artificial Sequence
  artificial sequence
gctttaacgatcgggtgttcagctggagtccacgc

SEQ ID NO: 918 - DNA, 28 bp, Artificial Sequence
  artificial sequence
tttgaaaaaggaatcaaaccctcaatca

SEQ ID NO: 919 - DNA, 35 bp, Artificial Sequence
  artificial sequence
ctgcaaggggtaatcaaagtagaggcgcggacttg

SEQ ID NO: 920 - DNA, 49 bp, Artificial Sequence
  artificial sequence
gcgattactcttcgaatccccaggtcttcaggaagaaccgtgacttcaa

SEQ ID NO: 921 - DNA, 42 bp, Artificial Sequence
  artificial sequence
agttgggtactaatagcataaagctaaattatttccgataaa

SEQ ID NO: 922 - DNA, 35 bp, Artificial Sequence
  artificial sequence
taaaataaccttgctgaacctacgctcaacagtgc

SEQ ID NO: 923 - DNA, 35 bp, Artificial Sequence
  artificial sequence
gtgagaggcttttgagggtttggaagggacagttc

SEQ ID NO: 924 - DNA, 35 bp, Artificial Sequence
  artificial sequence
tcagtacggctgagaacgaggcactggttgcgggc

SEQ ID NO: 925 - DNA, 49 bp, Artificial Sequence
  artificial sequence
ggaaacaatatgattcattgcctgagagatcgtaaggataaagcctcag

SEQ ID NO: 926 - DNA, 42 bp, Artificial Sequence
  artificial sequence
cctcaccgagagatattcatctaaggctaattgggcttgaga

SEQ ID NO: 927 - DNA, 35 bp, Artificial Sequence
  artificial sequence
acgggaagctgataagatctacaaaggctcatatg

SEQ ID NO: 928 - DNA, 42 bp, Artificial Sequence
  artificial sequence
tcatcggaaacaggcctcgttgtcagagggtaattaaaaggt

SEQ ID NO: 929 - DNA, 36 bp, Artificial Sequence
  artificial sequence
aataccacaaagctatttcaactttaattggacata

SEQ ID NO: 930 - DNA, 49 bp, Artificial Sequence
  artificial sequence
taaataaatttggcaaatcaacagttgataccgacgcgagaaaaacaat

SEQ ID NO: 931 - DNA, 40 bp, Artificial Sequence
  artificial sequence
caatttgcccgaactcgacaattttttacctgcaattttt

SEQ ID NO: 932 - DNA, 42 bp, Artificial Sequence
  artificial sequence
aaacaggtagaaagagactttgacctgccctgatagcttacg

SEQ ID NO: 933 - DNA, 49 bp, Artificial Sequence
  artificial sequence
gttattaattttaattatcaggaggtgatcgccatgcccaatgcgccgc

SEQ ID NO: 934 - DNA, 42 bp, Artificial Sequence
  artificial sequence
tcataggagaacgggtcctgatccaaatacggtaccaagttt

SEQ ID NO: 935 - DNA, 42 bp, Artificial Sequence
  artificial sequence
taccgacgagcgctgtataacgtgctttaggccgacgtcaaa

SEQ ID NO: 936 - DNA, 41 bp, Artificial Sequence
  artificial sequence
aaaaaatcccgtatggtttagctcattggccagatagaacg

SEQ ID NO: 937 - DNA, 42 bp, Artificial Sequence
  artificial sequence
aaaaaagccagcagttgggcggttaataatttagggtcccgg

SEQ ID NO: 938 - DNA, 49 bp, Artificial Sequence
  artificial sequence
ggcggccagtagtatgccctggtctcgtgtctggtgaaggtatggtttg

SEQ ID NO: 939 - DNA, 28 bp, Artificial Sequence
  artificial sequence
aacgtaacattcaagaagaaaaatctac

SEQ ID NO: 940 - DNA, 42 bp, Artificial Sequence
  artificial sequence
cagtgaaagttgagaaacgaactaacggtttgccgccgcaca

SEQ ID NO: 941 - DNA, 35 bp, Artificial Sequence
  artificial sequence
tatactgaattaccgaaacagtacataattaagac

SEQ ID NO: 942 - DNA, 56 bp, Artificial Sequence
  artificial sequence
ttatactccttagaatccttgaccttgctagatttaaacaattgctttgaatgatg

SEQ ID NO: 943 - DNA, 35 bp, Artificial Sequence
  artificial sequence
accgaacgaaccataacccactatggttatagaaa

SEQ ID NO: 944 - DNA, 35 bp, Artificial Sequence
  artificial sequence
gcacatcagtccacatataaagaatacccaaaaga

SEQ ID NO: 945 - DNA, 42 bp, Artificial Sequence
  artificial sequence
cttcatcccgaactgaccaacatctttgcgggcgcgcggctg

SEQ ID NO: 946 - DNA, 35 bp, Artificial Sequence
  artificial sequence
atcttgatcaccgtgatagcagcctttaattattc

SEQ ID NO: 947 - DNA, 35 bp, Artificial Sequence
  artificial sequence
taaccagcagaagagccaacaaaagaaccgtgtga

SEQ ID NO: 948 - DNA, 42 bp, Artificial Sequence
  artificial sequence
ccggaaccaacggagcatcagtcccttagtagcaacagggag

SEQ ID NO: 949 - DNA, 35 bp, Artificial Sequence
  artificial sequence
aacactctttgaaaataggctggctgacatttggg

SEQ ID NO: 950 - DNA, 42 bp, Artificial Sequence
  artificial sequence
ggttgcgggccggaaattagagccagcacaggcgcgaggaca

SEQ ID NO: 951 - DNA, 35 bp, Artificial Sequence
  artificial sequence
aatccgcacccccagcgattaaagggaaaagagta

SEQ ID NO: 952 - DNA, 42 bp, Artificial Sequence
  artificial sequence
gcgcttttttctttttgaggaatattcgtgttaattgtatcg

SEQ ID NO: 953 - DNA, 21 bp, Artificial Sequence
  artificial sequence
ttaattgagtattacatcata

SEQ ID NO: 954 - DNA, 35 bp, Artificial Sequence
  artificial sequence
gtaaaggcgcactcaaccatccaccgacttgagcc

SEQ ID NO: 955 - DNA, 35 bp, Artificial Sequence
  artificial sequence
gcaaatcaaagacatgcgggagccccctgttttca

SEQ ID NO: 956 - DNA, 42 bp, Artificial Sequence
  artificial sequence
atgaggacatcgccagcttgctttcgagaccgccaaggtgta

SEQ ID NO: 957 - DNA, 28 bp, Artificial Sequence
  artificial sequence
attcttataacaactaaaacaatgatgg

SEQ ID NO: 958 - DNA, 35 bp, Artificial Sequence
  artificial sequence
cggctactgaaagtacagaatgccagaacgcgtac

SEQ ID NO: 959 - DNA, 42 bp, Artificial Sequence
  artificial sequence
tgtcactctgcattataagtgttatcctatcccaaacaagaa

SEQ ID NO: 960 - DNA, 35 bp, Artificial Sequence
  artificial sequence
agcgcaggcggccaataatttgctaaacctcgaat

SEQ ID NO: 961 - DNA, 35 bp, Artificial Sequence
  artificial sequence
gcgggccgcatcagcgcgcgggttttgcctaacga

SEQ ID NO: 962 - DNA, 42 bp, Artificial Sequence
  artificial sequence
aacgcgcctgtttatgtttaattaaaggactgtagccaatga

SEQ ID NO: 963 - DNA, 42 bp, Artificial Sequence
  artificial sequence
caactaatcagcggtgaggatccccgggttatccgaactaca

SEQ ID NO: 964 - DNA, 42 bp, Artificial Sequence
  artificial sequence
tccttatccaacaggcagattcatcgtaggaatcataagaac

SEQ ID NO: 965 - DNA, 35 bp, Artificial Sequence
  artificial sequence
aactttcaacagttaggaatttaccgtaaattgcg

SEQ ID NO: 966 - DNA, 49 bp, Artificial Sequence
  artificial sequence
tcgtaatcatggttctgtatgggatttttttcacgcaagccccgctttc

SEQ ID NO: 967 - DNA, 35 bp, Artificial Sequence
  artificial sequence
aaaacatcctgattctgtcttatcccatcagccat

SEQ ID NO: 968 - DNA, 49 bp, Artificial Sequence
  artificial sequence
aatcagtttaaaggattcataagggttgttagagccggaaccctaaagg

SEQ ID NO: 969 - DNA, 35 bp, Artificial Sequence
  artificial sequence
ccacagacagccctgggatagttgaaaacactctg

SEQ ID NO: 970 - DNA, 35 bp, Artificial Sequence
  artificial sequence
acgcctgacccatggcgaatagaatgcggcatcgt

SEQ ID NO: 971 - DNA, 49 bp, Artificial Sequence
  artificial sequence
aagtgttccctgagcaagcgggtgtccagatttgtagttttgcagacga

SEQ ID NO: 972 - DNA, 35 bp, Artificial Sequence
  artificial sequence
aagggaccctgagttacaattccgtcgatgaaaca

SEQ ID NO: 973 - DNA, 35 bp, Artificial Sequence
  artificial sequence
acactgagtttcgtaaaggaacggtcatgtcacgt

SEQ ID NO: 974 - DNA, 49 bp, Artificial Sequence
  artificial sequence
atgtattatttgccggccacctgattgcccccagcgcaaccaaattgtg

SEQ ID NO: 975 - DNA, 35 bp, Artificial Sequence
  artificial sequence
cacacgaccagtaccaagcaagccgtttcgaacct

SEQ ID NO: 976 - DNA, 32 bp, Artificial Sequence
  artificial sequence
tttatcgcacaaattttttcctgataacggat

SEQ ID NO: 977 - DNA, 35 bp, Artificial Sequence
  artificial sequence
aatattgcaaagacatcaaaacggcgaaaggtgcc

SEQ ID NO: 978 - DNA, 35 bp, Artificial Sequence
  artificial sequence
tccagagtcaggattagcgggggagaggtcacatt

SEQ ID NO: 979 - DNA, 35 bp, Artificial Sequence
  artificial sequence
tcaccgttaaacagattaaacgtcactgttgccct

SEQ ID NO: 980 - DNA, 35 bp, Artificial Sequence
  artificial sequence
gagggttgactgtcgtgccaggcgcgccgtcgctg

SEQ ID NO: 981 - DNA, 42 bp, Artificial Sequence
  artificial sequence
tagaaggttaccgcagctaaccggtttgtgccggttcgtcac

SEQ ID NO: 982 - DNA, 49 bp, Artificial Sequence
  artificial sequence
ggtattcttaccgcgattatttacattgagatagagattagtaccaacg

SEQ ID NO: 983 - DNA, 42 bp, Artificial Sequence
  artificial sequence
tatccagcttctttacccttctaatcgggtttggattcctga

SEQ ID NO: 984 - DNA, 35 bp, Artificial Sequence
  artificial sequence
ctggtaattgcgctcggccaaacgatccttaaagg

SEQ ID NO: 985 - DNA, 49 bp, Artificial Sequence
  artificial sequence
aactatctcacttgattctggcattccatccatcaatataatagcgata

SEQ ID NO: 986 - DNA, 49 bp, Artificial Sequence
  artificial sequence
ccttcacaagagaaggattttagcagcggttaacgactgttgtcccagt

SEQ ID NO: 987 - DNA, 42 bp, Artificial Sequence
  artificial sequence
aataacaggccttggcgaggcgttttagttattttcaccagt

SEQ ID NO: 988 - DNA, 35 bp, Artificial Sequence
  artificial sequence
aacgtcacgcgtttcccctgcccggaatccctcag

SEQ ID NO: 989 - DNA, 35 bp, Artificial Sequence
  artificial sequence
tgaggaaggttatccctaaattattttatttagaa

SEQ ID NO: 990 - DNA, 49 bp, Artificial Sequence
  artificial sequence
gcaccgtattgcagcgcgaaaagtaaaaactatcaagaacccatcgatg

SEQ ID NO: 991 - DNA, 32 bp, Artificial Sequence
  artificial sequence
attattcatttagcaaaaaaacaaattttaca

SEQ ID NO: 992 - DNA, 35 bp, Artificial Sequence
  artificial sequence
tgaattaacgtgccagacggtagccatgtttacca

SEQ ID NO: 993 - DNA, 42 bp, Artificial Sequence
  artificial sequence
ttattcaagtgcagagagtcgattaagacaggcggaatgaat

SEQ ID NO: 994 - DNA, 35 bp, Artificial Sequence
  artificial sequence
ccagcgcacggaaatcagcgttacttagaatttgt

SEQ ID NO: 995 - DNA, 35 bp, Artificial Sequence
  artificial sequence
gtaaagcactggcaataaaggtggcaactattaaa

SEQ ID NO: 996 - DNA, 42 bp, Artificial Sequence
  artificial sequence
actaaatttgacgggctatctgagttaataaaaataaataat

SEQ ID NO: 997 - DNA, 42 bp, Artificial Sequence
  artificial sequence
ccgagattggtttatacagggtcctgagattatttgaatctt

SEQ ID NO: 998 - DNA, 35 bp, Artificial Sequence
  artificial sequence
agttacagcgtcttagcaataaacaatacttatcc

SEQ ID NO: 999 - DNA, 35 bp, Artificial Sequence
  artificial sequence
gactccatacatactgattaagactcctggggtcg

SEQ ID NO: 1000 - DNA, 35 bp, Artificial Sequence
  artificial sequence
acgtcaacttataaaaaagggccgccgctcagtga

SEQ ID NO: 1001 - DNA, 49 bp, Artificial Sequence
  artificial sequence
aaataaacctaatttaaaacaggcggtcagaatcgtcaaatattaatgg

SEQ ID NO: 1002 - DNA, 35 bp, Artificial Sequence
  artificial sequence
tcgggagtcaggtttaacgtctatgtgagtgaata

SEQ ID NO: 1003 - DNA, 35 bp, Artificial Sequence
  artificial sequence
gaagataactttacaacttttccatattccagtat

SEQ ID NO: 1004 - DNA, 42 bp, Artificial Sequence
  artificial sequence
tttataagcttaataataagagcaagctatagccctacgagc

SEQ ID NO: 1005 - DNA, 28 bp, Artificial Sequence
  artificial sequence
aatgaaaaatgcagaaagtaattctgtc

SEQ ID NO: 1006 - DNA, 35 bp, Artificial Sequence
  artificial sequence
cgtggcgcgaaacaatgaaataaagccacaaatat

SEQ ID NO: 1007 - DNA, 35 bp, Artificial Sequence
  artificial sequence
agcaataggaaagcgaatagcgaacgtgagcctcc

SEQ ID NO: 1008 - DNA, 42 bp, Artificial Sequence
  artificial sequence
gagcgggagaaaggaaaatccagggcgattttttcacgagaa

SEQ ID NO: 1009 - DNA, 43 bp, Artificial Sequence
  artificial sequence
tttttagtaaataaaaaaggctttttttccaaaaggagccttg

SEQ ID NO: 1010 - DNA, 38 bp, Artificial Sequence
  artificial sequence
tttaacataaaaacagggccctttacagagagaatttt

SEQ ID NO: 1011 - DNA, 36 bp, Artificial Sequence
  artificial sequence
gaacaaaagaatcagagaagcgcattagacgggttt

SEQ ID NO: 1012 - DNA, 33 bp, Artificial Sequence
  artificial sequence
tttgatagccgaacaaagcttaagaagagagat

SEQ ID NO: 1013 - DNA, 33 bp, Artificial Sequence
  artificial sequence
aagaaacacccagcagatcaagattagttgttt

SEQ ID NO: 1014 - DNA, 37 bp, Artificial Sequence
  artificial sequence
acaccctcagacgacgacattttttataaacaacatg

SEQ ID NO: 1015 - DNA, 29 bp, Artificial Sequence
  artificial sequence
tttggaataagtttggaacaagctcataa

SEQ ID NO: 1016 - DNA, 33 bp, Artificial Sequence
  artificial sequence
tttctattttgcgattttttcaacaatataaag

SEQ ID NO: 1017 - DNA, 29 bp, Artificial Sequence
  artificial sequence
tttttgtcacaatcagctttgagacagga

SEQ ID NO: 1018 - DNA, 29 bp, Artificial Sequence
  artificial sequence
tttcataacgccaaacaatcattaccaag

SEQ ID NO: 1019 - DNA, 38 bp, Artificial Sequence
  artificial sequence
tttaccgaggaaacgcaatgagttaccagaaggaattt

SEQ ID NO: 1020 - DNA, 29 bp, Artificial Sequence
  artificial sequence
gaactcacagtcgggaaacgccaccattt

SEQ ID NO: 1021 - DNA, 30 bp, Artificial Sequence
  artificial sequence
tttagtaagagcaactgtttagactggttt

SEQ ID NO: 1022 - DNA, 47 bp, Artificial Sequence
  artificial sequence
ggaacctgcgtcaggattttacgagcacaatatcaaagtaagcattt

SEQ ID NO: 1023 - DNA, 30 bp, Artificial Sequence
  artificial sequence
tttacagtgcccgtaactcaggaggttttt

SEQ ID NO: 1024 - DNA, 50 bp, Artificial Sequence
  artificial sequence
aagaatttaccgaatatacaaatatctggtcagtactagaaaaagccttt

SEQ ID NO: 1025 - DNA, 30 bp, Artificial Sequence
  artificial sequence
ttttgcggaatcgtctagtcagaagcattt

SEQ ID NO: 1026 - DNA, 31 bp, Artificial Sequence
  artificial sequence
tttgagaatcatcttttttgtaccgcaataa

SEQ ID NO: 1027 - DNA, 29 bp, Artificial Sequence
  artificial sequence
tttaagcggaacgacgacagtaataggaa

SEQ ID NO: 1028 - DNA, 29 bp, Artificial Sequence
  artificial sequence
tttaaaaagattaagaggaagcattgctc

SEQ ID NO: 1029 - DNA, 30 bp, Artificial Sequence
  artificial sequence
tttccctcattttcacatagttagcgtttt

SEQ ID NO: 1030 - DNA, 36 bp, Artificial Sequence
  artificial sequence
agaggctgctcgtcgccagctggcgaccaatacttt

SEQ ID NO: 1031 - DNA, 52 bp, Artificial Sequence
  artificial sequence
tttgccactacgaaggcgggggtaaatgcgccgtcttaaacagcttgatttt

SEQ ID NO: 1032 - DNA, 45 bp, Artificial Sequence
  artificial sequence
gatgaacaaagaatccaccaacctaaaacgttttttaaagaggca

SEQ ID NO: 1033 - DNA, 36 bp, Artificial Sequence
  artificial sequence
gaaccggatttttttattcattacaattaccttttt

SEQ ID NO: 1034 - DNA, 40 bp, Artificial Sequence
  artificial sequence
tttatgcgattttaagaaccattgtgccaaatccggacaa

SEQ ID NO: 1035 - DNA, 30 bp, Artificial Sequence
  artificial sequence
ttttcaggacgttggctaatgcagatattt

SEQ ID NO: 1036 - DNA, 48 bp, Artificial Sequence
  artificial sequence
tttggatggctttagatttagtttttttttgaccattacaggcaattt

SEQ ID NO: 1037 - DNA, 36 bp, Artificial Sequence
  artificial sequence
ttttaggttgggttatataaaatcctttgagagact

SEQ ID NO: 1038 - DNA, 43 bp, Artificial Sequence
  artificial sequence
tatgcgtgccctttccccgatagtgttgttccagtttattttt

SEQ ID NO: 1039 - DNA, 38 bp, Artificial Sequence
  artificial sequence
tttattttaattcgcgtctcttttgataagaggtcttt

SEQ ID NO: 1040 - DNA, 27 bp, Artificial Sequence
  artificial sequence
tttagtgaattttaacctccggctttt

SEQ ID NO: 1041 - DNA, 37 bp, Artificial Sequence
  artificial sequence
tttaaaagggtgagaaaggccgattacgaggcatttt

SEQ ID NO: 1042 - DNA, 29 bp, Artificial Sequence
  artificial sequence
aagagaatagataagtattaaaccaattt

SEQ ID NO: 1043 - DNA, 57 bp, Artificial Sequence
  artificial sequence
gcttagaatcaataagatgaacagtacccatcaagaaaacaaaattaattacatttt

SEQ ID NO: 1044 - DNA, 30 bp, Artificial Sequence
  artificial sequence
ttttgtttagtatcataggcagaggcattt

SEQ ID NO: 1045 - DNA, 48 bp, Artificial Sequence
  artificial sequence
tttttttcgagccagaccttttatcaaaagctgagaagagtcaatttt

SEQ ID NO: 1046 - DNA, 33 bp, Artificial Sequence
  artificial sequence
tctccaagaattttgtcgtctttccagacgttt

SEQ ID NO: 1047 - DNA, 36 bp, Artificial Sequence
  artificial sequence
gagacagcaaacaagatgtgtaggtaaagattcttt

SEQ ID NO: 1048 - DNA, 43 bp, Artificial Sequence
  artificial sequence
ttttgatgcaaaaataagaatttttttaaacaccggaatcata

SEQ ID NO: 1049 - DNA, 33 bp, Artificial Sequence
  artificial sequence
gaacgagagagcttcgccatcaaaaattgcttt

SEQ ID NO: 1050 - DNA, 43 bp, Artificial Sequence
  artificial sequence
tttggcaaagaattttaaatgttttttcaatgcctgagtaaga

SEQ ID NO: 1051 - DNA, 38 bp, Artificial Sequence
  artificial sequence
tttttttgaagccttaaaacccgacttgcgggaggttt

SEQ ID NO: 1052 - DNA, 37 bp, Artificial Sequence
  artificial sequence
tttgcaccattaccaggtcatagcccccttattagcg

SEQ ID NO: 1053 - DNA, 36 bp, Artificial Sequence
  artificial sequence
ctgctcaaacaacattattgagacgcagaaacattt

SEQ ID NO: 1054 - DNA, 27 bp, Artificial Sequence
  artificial sequence
tttgtaatgggatagaccgggggtttt

SEQ ID NO: 1055 - DNA, 43 bp, Artificial Sequence
  artificial sequence
ttcaaagcggaagcagtaacaacccgtcggattctccgtgttt

SEQ ID NO: 1056 - DNA, 37 bp, Artificial Sequence
  artificial sequence
tttggaacaaacggcggcagaccgaacattgaccttt

SEQ ID NO: 1057 - DNA, 27 bp, Artificial Sequence
  artificial sequence
ttttttgttaaagcttctggtgccttt

SEQ ID NO: 1058 - DNA, 37 bp, Artificial Sequence
  artificial sequence
tttattgtataagcaaatatagcacgacgttgtattt

SEQ ID NO: 1059 - DNA, 30 bp, Artificial Sequence
  artificial sequence
tttggtggagccgccgtgaagggatagttt

SEQ ID NO: 1060 - DNA, 27 bp, Artificial Sequence
  artificial sequence
tttgtaaacggtgccattcgccatttt

SEQ ID NO: 1061 - DNA, 33 bp, Artificial Sequence
  artificial sequence
cggcaccattcgcagcaactaaattaatatttt

SEQ ID NO: 1062 - DNA, 37 bp, Artificial Sequence
  artificial sequence
tttgcggatcaaactatgaagggtaaagttaaacttt

SEQ ID NO: 1063 - DNA, 43 bp, Artificial Sequence
  artificial sequence
tttgatgctgattgccgttcaccagaacgtttagtgtaaattt

SEQ ID NO: 1064 - DNA, 33 bp, Artificial Sequence
  artificial sequence
agaaagcacggtgttggggcgcgttaaattttt

SEQ ID NO: 1065 - DNA, 36 bp, Artificial Sequence
  artificial sequence
ctgaaaataccaaaaacattatgacccaggaagttt

SEQ ID NO: 1066 - DNA, 27 bp, Artificial Sequence
  artificial sequence
ttttcaggctgcgcagcatcagatttt

SEQ ID NO: 1067 - DNA, 33 bp, Artificial Sequence
  artificial sequence
gttgatattttgagaattaatgccggagagttt

SEQ ID NO: 1068 - DNA, 27 bp, Artificial Sequence
  artificial sequence
tttaaacgacggccatcggtggtgttt

SEQ ID NO: 1069 - DNA, 27 bp, Artificial Sequence
  artificial sequence
tttttctgccagaaagcctggggtttt

SEQ ID NO: 1070 - DNA, 37 bp, Artificial Sequence
  artificial sequence
tttttcgcgtccgtgagcctcccaacatacgagcttt

SEQ ID NO: 1071 - DNA, 43 bp, Artificial Sequence
  artificial sequence
tttcgtaaaacagaaataaagattatcatgaattatacaccgc

SEQ ID NO: 1072 - DNA, 27 bp, Artificial Sequence
  artificial sequence
tttctctcacggaaaaccggcaaattt

SEQ ID NO: 1073 - DNA, 44 bp, Artificial Sequence
  artificial sequence
tttgcctaatgagtgcagccataaattaaaagaatacgtggttt

SEQ ID NO: 1074 - DNA, 30 bp, Artificial Sequence
  artificial sequence
tttgtctttaatgcgctgcaacagtgcttt

SEQ ID NO: 1075 - DNA, 27 bp, Artificial Sequence
  artificial sequence
tttacgggcaacagcgagtaaaagttt

SEQ ID NO: 1076 - DNA, 27 bp, Artificial Sequence
  artificial sequence
tttggtagctatatcagaaaagccttt

SEQ ID NO: 1077 - DNA, 43 bp, Artificial Sequence
  artificial sequence
ttttgtttgagattgagggaggcagcagcaatccgcctccgtg

SEQ ID NO: 1078 - DNA, 27 bp, Artificial Sequence
  artificial sequence
ttttccgaaatcggcaagggaagattt

SEQ ID NO: 1079 - DNA, 29 bp, Artificial Sequence
  artificial sequence
tttcagggcgtgttagcaaacgtagaaaa

SEQ ID NO: 1080 - DNA, 29 bp, Artificial Sequence
  artificial sequence
tattacgcagtaatggcccactacgtttt

SEQ ID NO: 1081 - DNA, 29 bp, Artificial Sequence
  artificial sequence
tttgaaccatcacccaaatcaagtttttt

SEQ ID NO: 1082 - DNA, 27 bp, Artificial Sequence
  artificial sequence
tttaagcgaaagagcaaatgaaaattt

SEQ ID NO: 1083 - DNA, 38 bp, Artificial Sequence
  artificial sequence
tttacggcagcaccgtcgaaaccgcaagaatgccattt

SEQ ID NO: 1084 - DNA, 27 bp, Artificial Sequence
  artificial sequence
tttagtctgttagaatggctattattt

SEQ ID NO: 1085 - DNA, 37 bp, Artificial Sequence
  artificial sequence
tgcaacaggaaattttttaacgctcatggaaaagata

SEQ ID NO: 1086 - DNA, 36 bp, Artificial Sequence
  artificial sequence
tgaaatggcccaatagcaagcaaatctacctacttt

SEQ ID NO: 1087 - DNA, 36 bp, Artificial Sequence
  artificial sequence
tttattttgacgctcaatcgtcaaagcgtccgttgt

SEQ ID NO: 1088 - DNA, 27 bp, Artificial Sequence
  artificial sequence
tttgccgggttcttcaccagtgagttt

SEQ ID NO: 1089 - DNA, 43 bp, Artificial Sequence
  artificial sequence
cgaactgagggcgcaccacaccgacattcaacctggtggtttt

SEQ ID NO: 1090 - DNA, 38 bp, Artificial Sequence
  artificial sequence
ttttaatgtttttttttttttaacaatttcattagtaa

SEQ ID NO: 1091 - DNA, 27 bp, Artificial Sequence
  artificial sequence
tttcacgctgagagctctcaatagttt

SEQ ID NO: 1092 - DNA, 27 bp, Artificial Sequence
  artificial sequence
tttagccagcggcgtattgggcgcttt

SEQ ID NO: 1093 - DNA, 29 bp, Artificial Sequence
  artificial sequence
tttctaatagattagagccgatcttctga

SEQ ID NO: 1094 - DNA, 33 bp, Artificial Sequence
  artificial sequence
tttataatacatttgaggagttaattcaagggc

SEQ ID NO: 1095 - DNA, 43 bp, Artificial Sequence
  artificial sequence
agtaacaaattgcgttctgtaaatcgtcgctatatttgcattt

SEQ ID NO: 1096 - DNA, 46 bp, Artificial Sequence
  artificial sequence
tttgcggaacaaagaattttttaccaccagagggttagaacctttt

SEQ ID NO: 1097 - DNA, 50 bp, Artificial Sequence
  artificial sequence
tttaccatatcaaaatttaattaattttctctgaataatggaaaggagcg

SEQ ID NO: 1098 - DNA, 43 bp, Artificial Sequence
  artificial sequence
ttccacatcacagtagtgagaatagcacgcgtgcctgttcttt

SEQ ID NO: 1099 - DNA, 54 bp, Artificial Sequence
  artificial sequence
gttgtgtacatcgctcattataccagttttgacgatccatcgcccagggcgctg

SEQ ID NO: 1100 - DNA, 62 bp, Artificial Sequence
  artificial sequence
aataacgagaaacgcaaagacaccacttttgatcggtccgcggtgcggggaacgccactggc

SEQ ID NO: 1101 - DNA, 50 bp, Artificial Sequence
  artificial sequence
aagtttgagcccgcccactcgtgcaattttacagacaaatcaccagtatt

SEQ ID NO: 1102 - DNA, 40 bp, Artificial Sequence
  artificial sequence
tttagaattaactgattttcgtagacagcaccgcgtgcgt

SEQ ID NO: 1103 - DNA, 64 bp, Artificial Sequence
  artificial sequence
ggcgttatccaatctactatatgtaaatgctttctgagtcgctctctcgcaacagaggtacctc

SEQ ID NO: 1104 - DNA, 54 bp, Artificial Sequence
  artificial sequence
gtgacgatagaggtcatcatatccttttaacgatctaaagtttcatagctgttt

SEQ ID NO: 1105 - DNA, 59 bp, Artificial Sequence
  artificial sequence
taacacgaaagcaccggttaagcaaaattttttcagctatagcaggggagctcattttc

SEQ ID NO: 1106 - DNA, 38 bp, Artificial Sequence
  artificial sequence
ttttagtaccgccacttttaacattagcactcacgacc

SEQ ID NO: 1107 - DNA, 39 bp, Artificial Sequence
  artificial sequence
cagtttgaggggttgcatcttttgtttacaagcggtggc

SEQ ID NO: 1108 - DNA, 54 bp, Artificial Sequence
  artificial sequence
tcacccttagatacgtgcgaaaaattttatagcgtaagggggatgtgcatccaa

SEQ ID NO: 1109 - DNA, 44 bp, Artificial Sequence
  artificial sequence
tatgcggcgattgagtcaggtttttcgatagtatacgtaatttt

SEQ ID NO: 1110 - DNA, 44 bp, Artificial Sequence
  artificial sequence
ttagcaagtatgagacactaattttttcaccgcgccacatagca

SEQ ID NO: 1111 - DNA, 42 bp, Artificial Sequence
  artificial sequence
atgcggccttcgtcgtttcagggtggttttccccatcacttt

SEQ ID NO: 1112 - DNA, 42 bp, Artificial Sequence
  artificial sequence
atgcggccttcgtcgtttccatcccacaggcgaaaatccttt

SEQ ID NO: 1113 - DNA, 52 bp, Artificial Sequence
  artificial sequence
atgcggccttcgtcgtttccaaaaactgtaatactttcaagctttcagattt

SEQ ID NO: 1114 - DNA, 42 bp, Artificial Sequence
  artificial sequence
atgcggccttcgtcgtttcgcggtccgaaaaccgtctatttt

SEQ ID NO: 1115 - DNA, 53 bp, Artificial Sequence
  artificial sequence
atgcggccttcgtcgtttcacgctgcgcgtaacctggcaagtgtagcggtttt

SEQ ID NO: 1116 - DNA, 51 bp, Artificial Sequence
  artificial sequence
atgcggccttcgtcgtttcggaagcataaagtgtcaccagtacactcacaa

SEQ ID NO: 1117 - DNA, 42 bp, Artificial Sequence
  artificial sequence
atgcggccttcgtcgtttggaaaccaggcacctacctgcttt

SEQ ID NO: 1118 - DNA, 52 bp, Artificial Sequence
  artificial sequence
atgcggccttcgtcgtttatctaaagcatctctttaggagcactaacaattt

SEQ ID NO: 1119 - DNA, 50 bp, Artificial Sequence
  artificial sequence
atgcggccttcgtcgtttcacagacaatatttgaaaccaatcaatgaccg

SEQ ID NO: 1120 - DNA, 33 bp, Artificial Sequence
  artificial sequence
agccagaatctaaacaggtcagacgattggcca

SEQ ID NO: 1121 - DNA, 38 bp, Artificial Sequence
  artificial sequence
gcgcagtaccgttccaggccacattgacggcaaataaa

SEQ ID NO: 1122 - DNA, 35 bp, Artificial Sequence
  artificial sequence
agagccgccgccagtcttttccggaaccgcggaaa

SEQ ID NO: 1123 - DNA, 32 bp, Artificial Sequence
  artificial sequence
ccctcagagccgccccaccacataatcaaaat

SEQ ID NO: 1124 - DNA, 22 bp, Artificial Sequence
  artificial sequence
gaaccaccaccccaccctcaga

SEQ ID NO: 1125 - DNA, 32 bp, Artificial Sequence
  artificial sequence
agagaccctcacctcagagccttgatattcac